European Patent Application EP 4 617 368 A1, published September 17, 2025. Title: Advanced recombinant vector based on cucumber mosaic virus. Applicant: KT&G CORPORATION. Application KR. The sequence listing filed with the application follows.

SEQUENCE LISTING (10 sequences)

SEQ ID NO: 1 - DNA, 11926 bp, synthetic construct
  source 1..11926: mol_type = other DNA
gtaatcttaccactgtgtgtgtgtgtgtgtgtgtgtcgcgtcgtgtcgtgtcgtgttgtccgcacatttgagtcgtgctgtccgcaccttttctttcagtgtgttagaatacccgaggcatggctttccaaggtaccagcaggactttaactcaacagtcctcagcggctacgtctgacgaacttcaaaagatattatttagccctgaagccattaagaaaatggctgctgagtgtgacctaggccggcatcattggatgcgagctgataatgctatttcagtccggcccctcgttcccgaagtaacccacggtcgcattgtttctttctttaagtctgggtatgatgctggtgaattgtgctctaaaggatacatgagcgtccctcaagtgttgtgtgctgttactcgaacagtttccactgatgctgaagggtctctgagaatttacctagctgacttaggcgacaaggaattatctcccatagataagcaatgtgtcacattacataaccatgatctccccgctttagtgtctttccaaccgacgtatgattgtcctatggagacagttgggaatcggaagcggtgttttgctgtcgttattgagagacatggttacgttgggtataccggcaccacagctagcgtgtgtagtaattggcaagcacggttttcttctaagaataacaactacactcatatcgcagctgggaagactctagtactgccattcaatagattagctgagcaaacgaaaccgtcagccgtcgctcgcctattgaagtcgcaattgaataacatagaagcttcgcaatacgttttgacggattcgaagatcaatcagaatgcgcgcagtgagtccgaggaattaaatgttgagagccctcccgccgcaatcgggagttcttccgcgtcccgcttcgaaaccttcagaccgcaggtggttaacggtctttagattttcgtcgcgtattagtatataagtatgtgtgagtctgtacataatactatatctatagtgtcctgtgtgagttgatacagtagacaactgtgacgcgatgtcgtgttgagaagggaacacatctggttctagtaagccacatcattagttttgaggttcaattcctcttactccctgttgtgccccttactttttcatggatgcttctccacgaaattgcgtttcgtctactagatcaaggagtgtttgtgttgtgattttctctttgtgttgtagatatttgagtcgagtcatggacaaatctgaaactagtacgcgtgactacaaggacgacgatgacaaggcagattataaagatgatgacgataaacatcatcaccatcaccactgaacctgtgttttccagaaccctccctccgattctgtggcgggagctgagttggtagtgttgctataaactacctgaagtcactaaacgctatgcggtgaacgggttgtccatccagcttacggctaaaatggtcagtcgtggagaaatccacgccagtagacttacaagtctctgaggtgcctttgaaaccatctcctaggtttcttcggaaggacttcggtccgtgtacttctagcacaagatgctagtttagagtacgggcatcccccattttttttaatggggtctctcaaaggagaccaggatccgataccctgtcaccggatgtgttttccggtctgatgagtccgtgaggacgaaacaggactgtcctgcaggagctcgaattcggtacgctgaaatcaccagtctctctctacaaatctatctctctctattttctccataaataatgtgtgagtagtttccgataaggaaattagggttcttatagggtttcgtcatgtgttgagcatataagaaacccttagtatgtatttgtatttgtaaaatacttctatcaataaaatttctaattcctaaaaccaaaatcagtactaaatcagatccccaattcactggccgtcgttttacaacgtcgtgactgggaaaaccctggcgttacccaacttaatcgccttgcagcacatccccctttcgccagtggcactggccgtcgttttacaacgtcgtgactgggaaaaccctggcgttacccaacttaatcgccttgcagcacatccccctttcgccagctggcgtaatagcgaagaggcccgcaccgatcgcccttcccaacagttgcgcagcctgaatggcgaatgctagagcagcttgagcttggatcagattgtcgtttcccgccttcagtttaaactatcagtgtttgacaggatatattggcgggtaaacctaagagaaaagagcgtttattagaataacggatatttaaaagggcgtgaaaaggtttatccgttcgtccatttgtatgtgcatgccaaccacagggttcccctcgggatcaaagtactttgatccaacccctccgctgctatagtgcagtcggcttctgacgttcagtgcagccgtcttctgaaaacgacatgtcgcacaagtcctaagttacgcgacaggctgccgccctgcccttttcctggcgttttcttgtcgcgtgttttagtcgcataaagtagaatacttgcgactagaaccggagacattacgccatgaacaagagcgccgccgctggcctgctgggctatgcccgcgtcagcaccgacgaccaggacttgaccaaccaacgggccgaactgcacgcggccggctgcaccaagctgttttccgagaagatcaccggcaccaggcgcgaccgcccggagctggccaggatgcttgaccacctacgccctggcgacgttgtgacagtgaccaggctagaccgcctggcccgcagcacccgcgacctactggacattgccgagcgcatccaggaggccggcgcgggcctgcgtagcctggcagagccgtgggccgacaccaccacgccggccggccgcatggtgttgaccgtgttcgccggcattgccgagttcgagcgttccctaatcatcgaccgcacccggagcgggcgcgaggccgccaaggcccgaggcgtgaagtttggcccccgccctaccctcaccccggcacagatcgcgcacgcccgcgagctgatcgaccaggaaggccgcaccgtgaaagaggcggctgcactgcttggcgtgcatcgctcgaccctgtaccgcgcacttgagcgcagcgaggaagtgacgcccaccgaggccaggcggcgcggtgccttccgtgaggacgcattgaccgaggccgacgccctggcggccgccgagaatgaacgccaagaggaacaagcatgaaaccgcaccaggacggccaggacgaaccgtttttcattaccgaagagatcgaggcggagatgatcgcggccgggtacgtgttcgagccgcccgcgcacgtctcaaccgtgcggctgcatgaaatcctggccggtttgtctgatgccaagctggcggcctggccggccagcttggccgctgaagaaaccgagcgccgccgtctaaaaaggtgatgtgtatttgagtaaaacagcttgcgtcatgcggtcgctgcgtatatgatgcgatgagtaaataaacaaatacgcaaggggaacgcatgaaggttatcgctgtacttaaccagaaaggcgggtcaggcaagacgaccatcgcaacccatctagcccgcgccctgcaactcgccggggccgatgttctgttagtcgattccgatccccagggcagtgcccgcgattgggcggccgtgcgggaagatcaaccgctaaccgttgtcggcatcgaccgcccgacgattgaccgcgacgtgaaggccatcggccggcgcgacttcgtagtgatcgacggagcgccccaggcggcggacttggctgtgtccgcgatcaaggcagccgacttcgtgctgattccggtgcagccaagcccttacgacatatgggccaccgccgacctggtggagctggttaagcagcgcattgaggtcacggatggaaggctacaagcggcctttgtcgtgtcgcgggcgatcaaaggcacgcgcatcggcggtgaggttgccgaggcgctggccgggtacgagctgcccattcttgagtcccgtatcacgcagcgcgtgagctacccaggcactgccgccgccggcacaaccgttcttgaatcagaacccgagggcgacgctgcccgcgaggtccaggcgctggccgctgaaattaaatcaaaactcatttgagttaatgaggtaaagagaaaatgagcaaaagcacaaacacgctaagtgccggccgtccgagcgcacgcagcagcaaggctgcaacgttggccagcctggcagacacgccagccatgaagcgggtcaactttcagttgccggcggaggatcacaccaagctgaagatgtacgcggtacgccaaggcaagaccattaccgagctgctatctgaatacatcgcgcagctaccagagtaaatgagcaaatgaataaatgagtagatgaattttagcggctaaaggaggcggcatggaaaatcaagaacaaccaggcaccgacgccgtggaatgccccatgtgtggaggaacgggcggttggccaggcgtaagcggctgggttgtctgccggccctgcaatggcactggaacccccaagcccgaggaatcggcgtgacggtcgcaaaccatccggcccggtacaaatcggcgcggcgctgggtgatgacctggtggagaagttgaaggccgcgcaggccgcccagcggcaacgcatcgaggcagaagcacgccccggtgaatcgtggcaagcggccgctgatcgaatccgcaaagaatcccggcaaccgccggcagccggtgcgccgtcgattaggaagccgcccaagggcgacgagcaaccagattttttcgttccgatgctctatgacgtgggcacccgcgatagtcgcagcatcatggacgtggccgttttccgtctgtcgaagcgtgaccgacgagctggcgaggtgatccgctacgagcttccagacgggcacgtagaggtttccgcagggccggccggcatggccagtgtgtgggattacgacctggtactgatggcggtttcccatctaaccgaatccatgaaccgataccgggaagggaagggagacaagcccggccgcgtgttccgtccacacgttgcggacgtactcaagttctgccggcgagccgatggcggaaagcagaaagacgacctggtagaaacctgcattcggttaaacaccacgcacgttgccatgcagcgtacgaagaaggccaagaacggccgcctggtgacggtatccgagggtgaagccttgattagccgctacaagatcgtaaagagcgaaaccgggcggccggagtacatcgagatcgagctagctgattggatgtaccgcgagatcacagaaggcaagaacccggacgtgctgacggttcaccccgattactttttgatcgatcccggcatcggccgttttctctaccgcctggcacgccgcgccgcaggcaaggcagaagccagatggttgttcaagacgatctacgaacgcagtggcagcgccggagagttcaagaagttctgtttcaccgtgcgcaagctgatcgggtcaaatgacctgccggagtacgatttgaaggaggaggcggggcaggctggcccgatcctagtcatgcgctaccgcaacctgatcgagggcgaagcatccgccggttcctaatgtacggagcagatgctagggcaaattgccctagcaggggaaaaaggtcgaaaaggtctctttcctgtggatagcacgtacattgggaacccaaagccgtacattgggaaccggaacccgtacattgggaacccaaagccgtacattgggaaccggtcacacatgtaagtgactgatataaaagagaaaaaaggcgatttttccgcctaaaactctttaaaacttattaaaactcttaaaacccgcctggcctgtgcataactgtctggccagcgcacagccgaagagctgcaaaaagcgcctacccttcggtcgctgcgctccctacgccccgccgcttcgcgtcggcctatcgcggccgctggccgctcaaaaatggctggcctacggccaggcaatctaccagggcgcggacaagccgcgccgtcgccactcgaccgccggcgcccacatcaaggcaccctgcctcgcgcgtttcggtgatgacggtgaaaacctctgacacatgcagctcccggagacggtcacagcttgtctgtaagcggatgccgggagcagacaagcccgtcagggcgcgtcagcgggtgttggcgggtgtcggggcgcagccatgacccagtcacgtagcgatagcggagtgtatactggcttaactatgcggcatcagagcagattgtactgagagtgcaccatatgcggtgtgaaataccgcacagatgcgtaaggagaaaataccgcatcaggcgctcttccgcttcctcgctcactgactcgctgcgctcggtcgttcggctgcggcgagcggtatcagctcactcaaaggcggtaatacggttatccacagaatcaggggataacgcaggaaagaacatgtgagcaaaaggccagcaaaaggccaggaaccgtaaaaaggccgcgttgctggcgtttttccataggctccgcccccctgacgagcatcacaaaaatcgacgctcaagtcagaggtggcgaaacccgacaggactataaagataccaggcgtttccccctggaagctccctcgtgcgctctcctgttccgaccctgccgcttaccggatacctgtccgcctttctcccttcgggaagcgtggcgctttctcatagctcacgctgtaggtatctcagttcggtgtaggtcgttcgctccaagctgggctgtgtgcacgaaccccccgttcagcccgaccgctgcgccttatccggtaactatcgtcttgagtccaacccggtaagacacgacttatcgccactggcagcagccactggtaacaggattagcagagcgaggtatgtaggcggtgctacagagttcttgaagtggtggcctaactacggctacactagaaggacagtatttggtatctgcgctctgctgaagccagttaccttcggaaaaagagttggtagctcttgatccggcaaacaaaccaccgctggtagcggtggtttttttgtttgcaagcagcagattacgcgcagaaaaaaaggatctcaagaagatcctttgatcttttctacggggtctgacgctcagtggaacgaaaactcacgttaagggattttggtcatgcattctaggtactaaaacaattcatccagtaaaatataatattttattttctcccaatcaggcttgatccccagtaagtcaaaaaatagctcgacatactgttcttccccgatatcctccctgatcgaccggacgcagaaggcaatgtcataccacttgtccgccctgccgcttctcccaagatcaataaagccacttactttgccatctttcacaaagatgttgctgtctcccaggtcgccgtgggaaaagacaagttcctcttcgggcttttccgtctttaaaaaatcatacagctcgcgcggatctttaaatggagtgtcttcttcccagttttcgcaatccacatcggccagatcgttattcagtaagtaatccaattcggctaagcggctgtctaagctattcgtatagggacaatccgatatgtcgatggagtgaaagagcctgatgcactccgcatacagctcgataatcttttcagggctttgttcatcttcatactcttccgagcaaaggacgccatcggcctcactcatgagcagattgctccagccatcatgccgttcaaagtgcaggacctttggaacaggcagctttccttccagccatagcatcatgtccttttcccgttccacatcataggtggtccctttataccggctgtccgtcatttttaaatataggttttcattttctcccaccagcttatataccttagcaggagacattccttccgtatcttttacgcagcggtatttttcgatcagttttttcaattccggtgatattctcattttagccatttattatttccttcctcttttctacagtatttaaagataccccaagaagctaattataacaagacgaactccaattcactgttccttgcattctaaaaccttaaataccagaaaacagctttttcaaagttgttttcaaagttggcgtataacatagtatcgacggagccgattttgaaaccgcggtgatcacaggcagcaacgctctgtcatcgttacaatcaacatgctaccctccgcgagatcatccgtgtttcaaacccggcagcttagttgccgttcttccgaatagcatcggtaacatgagcaaagtctgccgccttacaacggctctcccgctgacgccgtcccggactgatgggctgcctgtatcgagtggtgattttgtgccgagctgccggtcggggagctgttggctggctggtggcaggatatattgtggtgtaaacaaattgacgcttagacaacttaataacacattgcggacgtttttaatgtactgaattaacgccgaattaattcgggggatctggattttagtactggattttggttttaggaattagaaattttattgatagaagtattttacaaatacaaatacatactaagggtttcttatatgctcaacacatgagcgaaaccctataggaaccctaattcccttatctgggaactactcacacattattatggagaaactcgagcttgtcgatcgacagatccggtcggcatctactctatttctttgccctcggacgagtgctggggcgtcggtttccactatcggcgagtacttctacacagccatcggtccagacggccgcgcttctgcgggcgatttgtgtacgcccgacagtcccggctccggatcggacgattgcgtcgcatcgaccctgcgcccaagctgcatcatcgaaattgccgtcaaccaagctctgatagagttggtcaagaccaatgcggagcatatacgcccggagtcgtggcgatcctgcaagctccggatgcctccgctcgaagtagcgcgtctgctgctccatacaagccaaccacggcctccagaagaagatgttggcgacctcgtattgggaatccccgaacatcgcctcgctccagtcaatgaccgctgttatgcggccattgtccgtcaggacattgttggagccgaaatccgcgtgcacgaggtgccggacttcggggcagtcctcggcccaaagcatcagctcatcgagagcctgcgcgacggacgcactgacggtgtcgtccatcacagtttgccagtgatacacatggggatcagcaatcgcgcatatgaaatcacgccatgtagtgtattgaccgattccttgcggtccgaatgggccgaacccgctcgtctggctaagatcggccgcagcgatcgcatccatagcctccgcgaccggttgtagaacagcgggcagttcggtttcaggcaggtcttgcaacgtgacaccctgtgcacggcgggagatgcaataggtcaggctctcgctaaactccccaatgtcaagcacttccggaatcgggagcgcggccgatgcaaagtgccgataaacataacgatctttgtagaaaccatcggcgcagctatttacccgcaggacatatccacgccctcctacatcgaagctgaaagcacgagattcttcgccctccgagagctgcatcaggtcggagacgctgtcgaacttttcgatcagaaacttctcgacagacgtcgcggtgagttcaggctttttcatatctcattgccccccgggatctgcgaaagctcgagagagatagatttgtagagagagactggtgatttcagcgtgtcctctccaaatgaaatgaacttccttatatagaggaaggtcttgcgaaggatagtgggattgtgcgtcatcccttacgtcagtggagatatcacatcaatccacttgctttgaagacgtggttggaacgtcttctttttccacgatgctcctcgtgggtgggggtccatctttgggaccactgtcggcagaggcatcttgaacgatagcctttcctttatcgcaatgatggcatttgtaggtgccaccttccttttctactgtccttttgatgaagtgacagatagctgggcaatggaatccgaggaggtttcccgatattaccctttgttgaaaagtctcaatagccctttggtcttctgagactgtatctttgatattcttggagtagacgagagtgtcgtgctccaccatgttatcacatcaatccacttgctttgaagacgtggttggaacgtcttctttttccacgatgctcctcgtgggtgggggtccatctttgggaccactgtcggcagaggcatcttgaacgatagcctttcctttatcgcaatgatggcatttgtaggtgccaccttccttttctactgtccttttgatgaagtgacagatagctgggcaatggaatccgaggaggtttcccgatattaccctttgttgaaaagtctcaatagccctttggtcttctgagactgtatctttgatattcttggagtagacgagagtgtcgtgctccaccatgttggcaagctgctctagccaatacgcaaaccgcctctccccgcgcgttggccgattcattaatgcagctggcacgacaggtttcccgactggaaagcgggcagtgagcgcaacgcaattaatgtgagttagctcactcattaggcaccccaggctttacactttatgcttccggctcgtatgttgtgtggaattgtgagcggataacaatttcacacaggaaacagctatgaccatgattacgaattctggcacgacaggtttcccgactggaaagcgggcagtgagcgcaacgcaattaatgtgagttagctcactcattaggcaccccaggctttacactttatgcttccggctcgtatgttgtgtggaattgtgagcggataacaatttcacacaggaaacagctatgaccatgattacgccaagcttgcatgcctgcaggtcaacatggtggagcacgacactctcgtctactccaagaatatcaaagatacagtctcagaagaccagagggctattgagacttttcaacaaagggtaatatcgggaaacctcctcggattccattgcccagctatctgtcacttcatcgaaaggacagtagaaaaggaagatggcttctacaaatgccatcattgcgataaaggaaaggctatcgttcaagatgcctctaccgacagtggtcccaaagatggacccccacccacgaggaacatcgtggaaaaagaagacgttccaaccacgtcttcaaagcaagtggattgatgtgatggtcaacatggtggagcacgacactctcgtctactccaagaatatcaaagatacagtctcagaagaccagagggctattgagacttttcaacaaagggtaatatcgggaaacctcctcggattccattgcccagctatctgtcacttcatcgaaaggacagtagaaaaggaagatggcttctacaaatgccatcattgcgataaaggaaaggctatcgttcaagatgcctctaccgacagtggtcccaaagatggacccccacccacgaggaacatcgtggaaaaagaagacgttccaaccacgtcttcaaagcaagtggattgatgtgatatctccactgacgtaagggatgacgcacaatcccactatccttcgcaagacccttcctctatataaggaagttcatttcatttggagaggcctgggtacctctaga

SEQ ID NO: 2 - DNA, 13691 bp, synthetic construct
  source 1..13691: mol_type = other DNA
gtttatttacaagagcgtacggttcaacccctgcctcccctgtaaaattccctagactttctagtttctttctttcctatggctttccctgcccccgctttctcattggccaatcttttgaatggtacttacggtgtcgacactcccgaggaagtggaacgtgtgcgatctgagcaacacgaagaggctgctgcggcttgtcgtaattacaagcctttacccgctgtggatgtcagcgagagtgtcacagaggatgcgcattccctccgaactccagacggagctccctttgaagaggtgtctgttgagctcgttacttttggtgctgaagattaccttggaaaatctgatgatgagctccttgtcgcttttgagacgatggtcaaacccatgtgtatcggacagttatggtgccctgcgtttaataaatgttcttttatttccagcattgctatggctagagctttgctgttggtacctagcacatccaaccgaaccatgaagtgttttgaagacctggtcgcggctatttacactaaatccgatttctattacgatgatgagtgtgaagctgacgacattcagataaatgtctcgtctcgcgatgtacccggttattctttcgaaccgtggtcccgaacatctggatttgaaccaccgcctatctgtgaggcgtgtgacatgatcatgtaccagtgcccgtgttttgattttaatgctttaaagaaatcgtgcgctgagaggactttcgctgatgactatgttattgaaggtttagatggtgttgttgacaatgcaactttgttgtctaatttaggcccatttttggtgcctgtgaagtgccaatacgagaaatgtccaacacccaccgtcgcgactcctccgagtttaaatcgtgctactgatcgtgttgatatcaatttagttcaatccatttgtgattccactctgcccacgcatagcaactacgatgactcttttcatcaagtgttcgtcgaaagcgctgattattctattgatctggatcatgttagacttcggcaatctgatctcattgcaaaaattccagaatcagggcatatgataccggttttaaataccgggagtggtcacaagagagtaggtacgacgaaggaggtccttacagcaatcaagaaacgtaatgctgacgttccagagctaggtgattccgttaatctgtccaggttgagtaaggctgtggctgagagatttttcatctcgtacattaatggcaactctttagccaccagcaactttgttaacgtcgttagcaatttccacgattacatggaaaaatggaagtcttcaggtctctcgtatgacgatcttccagatctgcatgctgagaatttgcagttttatgatcacatgataaaatctgatgtgaagcctgtcgttagcgacacattgaacattgacagaccggttccagctactataacgtatcacaagaaaggtataacctcccagttctcaccgttattcacagctctatttgagcgtttccagagatgccttcgagaacgtattattcttcctgttggaaagatttcatcccttgagatgtcaggatttgatgttaagaacaaacattgtctcgagatcgatttgtccaaattcgacaagtctcaaggtgaattccatttgatgattcaggaacacattttgaatggtctagggtgcccagctccgataactaagtggtggtgtgatttccacagattctcttacattagagaccgtagagctggtgttggtatgcctatcagtttccagagacgaactggtgatgcatttacctacttcggtaacaccatcgtcaccatggctgaatttgcatggtgttacgacaccgaccaattcgaaaagcttttattctcaggcgatgattctctaggattttcagtgcttccccctgttggcgatccgagtaagttcacaactcttttcaacatggaagctaaggtgatggagccagcagtaccatacatttgttcgaagtttctactctctgatgagttcggtaataccttttccgttccagatccattgcgcgaggttcagcggttaggaactaagaaaatcccctattccgacaatgacgaattcctgtttgctcacttcatgagctttgttgatcgattgaagtttttggaccgaatgactcagtcttgcatcgatcagctttcactcttctttgagttgaaatacaggaagtccggggcggaggctgccttgatgttaggcgcctttaagaaatataccgctaattttcagtcctacaaagaactctatttttcagatcgtcgtcagtgcgaattgatcaattcgtttagttgtgtagagttgaggattgagcgttcgagtttcattaagcagcgaaagaagaaagatggaattgaacgaaggcgcaatgacaaacgtcgaactccaactagcccgcatggtggaggcgaagagacagagacgaaggtctcacaagaagaatcgacgggaacgatgttacaaaagtcccagcgagagagcacgttcaaatctcagactgttccgcttcctaccgttctatcaagtagatggttcggaactgatagagatgtaccgccacgtgaacgtggcggaattgtccgagtctgagctgctaaacttcgatctcttgaagcttgcaggagatgttgagtcaaatccaggtccaacgcgtatgccaagcaaactcgcgctaatccaggaacttcccgaccgcattcaaacggcggtggaagcagccatgggaatgagctaccaagacgcaccgaacaacgtgcgcagggacctcgacaacctgcacgcttgcctaaacaaggcaaaactaacggtaagtcggatggtaacatcactgctggagaaacccagcgtggtggcatacctagagggaaaggcccccgaggaggcaaaaccaacactcgaagaacgcctccgaaagctggagctcagccacagccttccaacaaccggaagtgaccccccacccgcaaaactgtgaacgcgtactagtgactacaaggacgacgatgacaaggcagattataaagatgatgacgataaacatcatcaccatcaccactgaacccctccttcctttctccctccagttttctgaggcgggagctgagttggcagtattgctacaaactgtctgaagtcactaaacgttttacggtgaacgggttgtccatccagctaacggctaaaatggtcagtcgcggagaaatccacgccggagatttacaagtctctgaggcacctttgaaaccatctcctaggtttcttcggaaggacttcggtccgtgtacttctagcacaacgtgctagtttcagggtacgggtgccccccacttttgtggggcttcctgaaggagaccaggatccgataccctgtcaccggatgtgttttccggtctgatgagtccgtgaggacgaaacaggactgtcctgcaggagctcgaattcggtacgctgaaatcaccagtctctctctacaaatctatctctctctattttctccataaataatgtgtgagtagtttccgataaggaaattagggttcttatagggtttcgtcatgtgttgagcatataagaaacccttagtatgtatttgtatttgtaaaatacttctatcaataaaatttctaattcctaaaaccaaaatcagtactaaatcagatccccaattcactggccgtcgttttacaacgtcgtgactgggaaaaccctggcgttacccaacttaatcgccttgcagcacatccccctttcgccagtggcactggccgtcgttttacaacgtcgtgactgggaaaaccctggcgttacccaacttaatcgccttgcagcacatccccctttcgccagctggcgtaatagcgaagaggcccgcaccgatcgcccttcccaacagttgcgcagcctgaatggcgaatgctagagcagcttgagcttggatcagattgtcgtttcccgccttcagtttaaactatcagtgtttgacaggatatattggcgggtaaacctaagagaaaagagcgtttattagaataacggatatttaaaagggcgtgaaaaggtttatccgttcgtccatttgtatgtgcatgccaaccacagggttcccctcgggatcaaagtactttgatccaacccctccgctgctatagtgcagtcggcttctgacgttcagtgcagccgtcttctgaaaacgacatgtcgcacaagtcctaagttacgcgacaggctgccgccctgcccttttcctggcgttttcttgtcgcgtgttttagtcgcataaagtagaatacttgcgactagaaccggagacattacgccatgaacaagagcgccgccgctggcctgctgggctatgcccgcgtcagcaccgacgaccaggacttgaccaaccaacgggccgaactgcacgcggccggctgcaccaagctgttttccgagaagatcaccggcaccaggcgcgaccgcccggagctggccaggatgcttgaccacctacgccctggcgacgttgtgacagtgaccaggctagaccgcctggcccgcagcacccgcgacctactggacattgccgagcgcatccaggaggccggcgcgggcctgcgtagcctggcagagccgtgggccgacaccaccacgccggccggccgcatggtgttgaccgtgttcgccggcattgccgagttcgagcgttccctaatcatcgaccgcacccggagcgggcgcgaggccgccaaggcccgaggcgtgaagtttggcccccgccctaccctcaccccggcacagatcgcgcacgcccgcgagctgatcgaccaggaaggccgcaccgtgaaagaggcggctgcactgcttggcgtgcatcgctcgaccctgtaccgcgcacttgagcgcagcgaggaagtgacgcccaccgaggccaggcggcgcggtgccttccgtgaggacgcattgaccgaggccgacgccctggcggccgccgagaatgaacgccaagaggaacaagcatgaaaccgcaccaggacggccaggacgaaccgtttttcattaccgaagagatcgaggcggagatgatcgcggccgggtacgtgttcgagccgcccgcgcacgtctcaaccgtgcggctgcatgaaatcctggccggtttgtctgatgccaagctggcggcctggccggccagcttggccgctgaagaaaccgagcgccgccgtctaaaaaggtgatgtgtatttgagtaaaacagcttgcgtcatgcggtcgctgcgtatatgatgcgatgagtaaataaacaaatacgcaaggggaacgcatgaaggttatcgctgtacttaaccagaaaggcgggtcaggcaagacgaccatcgcaacccatctagcccgcgccctgcaactcgccggggccgatgttctgttagtcgattccgatccccagggcagtgcccgcgattgggcggccgtgcgggaagatcaaccgctaaccgttgtcggcatcgaccgcccgacgattgaccgcgacgtgaaggccatcggccggcgcgacttcgtagtgatcgacggagcgccccaggcggcggacttggctgtgtccgcgatcaaggcagccgacttcgtgctgattccggtgcagccaagcccttacgacatatgggccaccgccgacctggtggagctggttaagcagcgcattgaggtcacggatggaaggctacaagcggcctttgtcgtgtcgcgggcgatcaaaggcacgcgcatcggcggtgaggttgccgaggcgctggccgggtacgagctgcccattcttgagtcccgtatcacgcagcgcgtgagctacccaggcactgccgccgccggcacaaccgttcttgaatcagaacccgagggcgacgctgcccgcgaggtccaggcgctggccgctgaaattaaatcaaaactcatttgagttaatgaggtaaagagaaaatgagcaaaagcacaaacacgctaagtgccggccgtccgagcgcacgcagcagcaaggctgcaacgttggccagcctggcagacacgccagccatgaagcgggtcaactttcagttgccggcggaggatcacaccaagctgaagatgtacgcggtacgccaaggcaagaccattaccgagctgctatctgaatacatcgcgcagctaccagagtaaatgagcaaatgaataaatgagtagatgaattttagcggctaaaggaggcggcatggaaaatcaagaacaaccaggcaccgacgccgtggaatgccccatgtgtggaggaacgggcggttggccaggcgtaagcggctgggttgtctgccggccctgcaatggcactggaacccccaagcccgaggaatcggcgtgacggtcgcaaaccatccggcccggtacaaatcggcgcggcgctgggtgatgacctggtggagaagttgaaggccgcgcaggccgcccagcggcaacgcatcgaggcagaagcacgccccggtgaatcgtggcaagcggccgctgatcgaatccgcaaagaatcccggcaaccgccggcagccggtgcgccgtcgattaggaagccgcccaagggcgacgagcaaccagattttttcgttccgatgctctatgacgtgggcacccgcgatagtcgcagcatcatggacgtggccgttttccgtctgtcgaagcgtgaccgacgagctggcgaggtgatccgctacgagcttccagacgggcacgtagaggtttccgcagggccggccggcatggccagtgtgtgggattacgacctggtactgatggcggtttcccatctaaccgaatccatgaaccgataccgggaagggaagggagacaagcccggccgcgtgttccgtccacacgttgcggacgtactcaagttctgccggcgagccgatggcggaaagcagaaagacgacctggtagaaacctgcattcggttaaacaccacgcacgttgccatgcagcgtacgaagaaggccaagaacggccgcctggtgacggtatccgagggtgaagccttgattagccgctacaagatcgtaaagagcgaaaccgggcggccggagtacatcgagatcgagctagctgattggatgtaccgcgagatcacagaaggcaagaacccggacgtgctgacggttcaccccgattactttttgatcgatcccggcatcggccgttttctctaccgcctggcacgccgcgccgcaggcaaggcagaagccagatggttgttcaagacgatctacgaacgcagtggcagcgccggagagttcaagaagttctgtttcaccgtgcgcaagctgatcgggtcaaatgacctgccggagtacgatttgaaggaggaggcggggcaggctggcccgatcctagtcatgcgctaccgcaacctgatcgagggcgaagcatccgccggttcctaatgtacggagcagatgctagggcaaattgccctagcaggggaaaaaggtcgaaaaggtctctttcctgtggatagcacgtacattgggaacccaaagccgtacattgggaaccggaacccgtacattgggaacccaaagccgtacattgggaaccggtcacacatgtaagtgactgatataaaagagaaaaaaggcgatttttccgcctaaaactctttaaaacttattaaaactcttaaaacccgcctggcctgtgcataactgtctggccagcgcacagccgaagagctgcaaaaagcgcctacccttcggtcgctgcgctccctacgccccgccgcttcgcgtcggcctatcgcggccgctggccgctcaaaaatggctggcctacggccaggcaatctaccagggcgcggacaagccgcgccgtcgccactcgaccgccggcgcccacatcaaggcaccctgcctcgcgcgtttcggtgatgacggtgaaaacctctgacacatgcagctcccggagacggtcacagcttgtctgtaagcggatgccgggagcagacaagcccgtcagggcgcgtcagcgggtgttggcgggtgtcggggcgcagccatgacccagtcacgtagcgatagcggagtgtatactggcttaactatgcggcatcagagcagattgtactgagagtgcaccatatgcggtgtgaaataccgcacagatgcgtaaggagaaaataccgcatcaggcgctcttccgcttcctcgctcactgactcgctgcgctcggtcgttcggctgcggcgagcggtatcagctcactcaaaggcggtaatacggttatccacagaatcaggggataacgcaggaaagaacatgtgagcaaaaggccagcaaaaggccaggaaccgtaaaaaggccgcgttgctggcgtttttccataggctccgcccccctgacgagcatcacaaaaatcgacgctcaagtcagaggtggcgaaacccgacaggactataaagataccaggcgtttccccctggaagctccctcgtgcgctctcctgttccgaccctgccgcttaccggatacctgtccgcctttctcccttcgggaagcgtggcgctttctcatagctcacgctgtaggtatctcagttcggtgtaggtcgttcgctccaagctgggctgtgtgcacgaaccccccgttcagcccgaccgctgcgccttatccggtaactatcgtcttgagtccaacccggtaagacacgacttatcgccactggcagcagccactggtaacaggattagcagagcgaggtatgtaggcggtgctacagagttcttgaagtggtggcctaactacggctacactagaaggacagtatttggtatctgcgctctgctgaagccagttaccttcggaaaaagagttggtagctcttgatccggcaaacaaaccaccgctggtagcggtggtttttttgtttgcaagcagcagattacgcgcagaaaaaaaggatctcaagaagatcctttgatcttttctacggggtctgacgctcagtggaacgaaaactcacgttaagggattttggtcatgcattctaggtactaaaacaattcatccagtaaaatataatattttattttctcccaatcaggcttgatccccagtaagtcaaaaaatagctcgacatactgttcttccccgatatcctccctgatcgaccggacgcagaaggcaatgtcataccacttgtccgccctgccgcttctcccaagatcaataaagccacttactttgccatctttcacaaagatgttgctgtctcccaggtcgccgtgggaaaagacaagttcctcttcgggcttttccgtctttaaaaaatcatacagctcgcgcggatctttaaatggagtgtcttcttcccagttttcgcaatccacatcggccagatcgttattcagtaagtaatccaattcggctaagcggctgtctaagctattcgtatagggacaatccgatatgtcgatggagtgaaagagcctgatgcactccgcatacagctcgataatcttttcagggctttgttcatcttcatactcttccgagcaaaggacgccatcggcctcactcatgagcagattgctccagccatcatgccgttcaaagtgcaggacctttggaacaggcagctttccttccagccatagcatcatgtccttttcccgttccacatcataggtggtccctttataccggctgtccgtcatttttaaatataggttttcattttctcccaccagcttatataccttagcaggagacattccttccgtatcttttacgcagcggtatttttcgatcagttttttcaattccggtgatattctcattttagccatttattatttccttcctcttttctacagtatttaaagataccccaagaagctaattataacaagacgaactccaattcactgttccttgcattctaaaaccttaaataccagaaaacagctttttcaaagttgttttcaaagttggcgtataacatagtatcgacggagccgattttgaaaccgcggtgatcacaggcagcaacgctctgtcatcgttacaatcaacatgctaccctccgcgagatcatccgtgtttcaaacccggcagcttagttgccgttcttccgaatagcatcggtaacatgagcaaagtctgccgccttacaacggctctcccgctgacgccgtcccggactgatgggctgcctgtatcgagtggtgattttgtgccgagctgccggtcggggagctgttggctggctggtggcaggatatattgtggtgtaaacaaattgacgcttagacaacttaataacacattgcggacgtttttaatgtactgaattaacgccgaattaattcgggggatctggattttagtactggattttggttttaggaattagaaattttattgatagaagtattttacaaatacaaatacatactaagggtttcttatatgctcaacacatgagcgaaaccctataggaaccctaattcccttatctgggaactactcacacattattatggagaaactcgagcttgtcgatcgacagatccggtcggcatctactctatttctttgccctcggacgagtgctggggcgtcggtttccactatcggcgagtacttctacacagccatcggtccagacggccgcgcttctgcgggcgatttgtgtacgcccgacagtcccggctccggatcggacgattgcgtcgcatcgaccctgcgcccaagctgcatcatcgaaattgccgtcaaccaagctctgatagagttggtcaagaccaatgcggagcatatacgcccggagtcgtggcgatcctgcaagctccggatgcctccgctcgaagtagcgcgtctgctgctccatacaagccaaccacggcctccagaagaagatgttggcgacctcgtattgggaatccccgaacatcgcctcgctccagtcaatgaccgctgttatgcggccattgtccgtcaggacattgttggagccgaaatccgcgtgcacgaggtgccggacttcggggcagtcctcggcccaaagcatcagctcatcgagagcctgcgcgacggacgcactgacggtgtcgtccatcacagtttgccagtgatacacatggggatcagcaatcgcgcatatgaaatcacgccatgtagtgtattgaccgattccttgcggtccgaatgggccgaacccgctcgtctggctaagatcggccgcagcgatcgcatccatagcctccgcgaccggttgtagaacagcgggcagttcggtttcaggcaggtcttgcaacgtgacaccctgtgcacggcgggagatgcaataggtcaggctctcgctaaactccccaatgtcaagcacttccggaatcgggagcgcggccgatgcaaagtgccgataaacataacgatctttgtagaaaccatcggcgcagctatttacccgcaggacatatccacgccctcctacatcgaagctgaaagcacgagattcttcgccctccgagagctgcatcaggtcggagacgctgtcgaacttttcgatcagaaacttctcgacagacgtcgcggtgagttcaggctttttcatatctcattgccccccgggatctgcgaaagctcgagagagatagatttgtagagagagactggtgatttcagcgtgtcctctccaaatgaaatgaacttccttatatagaggaaggtcttgcgaaggatagtgggattgtgcgtcatcccttacgtcagtggagatatcacatcaatccacttgctttgaagacgtggttggaacgtcttctttttccacgatgctcctcgtgggtgggggtccatctttgggaccactgtcggcagaggcatcttgaacgatagcctttcctttatcgcaatgatggcatttgtaggtgccaccttccttttctactgtccttttgatgaagtgacagatagctgggcaatggaatccgaggaggtttcccgatattaccctttgttgaaaagtctcaatagccctttggtcttctgagactgtatctttgatattcttggagtagacgagagtgtcgtgctccaccatgttatcacatcaatccacttgctttgaagacgtggttggaacgtcttctttttccacgatgctcctcgtgggtgggggtccatctttgggaccactgtcggcagaggcatcttgaacgatagcctttcctttatcgcaatgatggcatttgtaggtgccaccttccttttctactgtccttttgatgaagtgacagatagctgggcaatggaatccgaggaggtttcccgatattaccctttgttgaaaagtctcaatagccctttggtcttctgagactgtatctttgatattcttggagtagacgagagtgtcgtgctccaccatgttggcaagctgctctagccaatacgcaaaccgcctctccccgcgcgttggccgattcattaatgcagctggcacgacaggtttcccgactggaaagcgggcagtgagcgcaacgcaattaatgtgagttagctcactcattaggcaccccaggctttacactttatgcttccggctcgtatgttgtgtggaattgtgagcggataacaatttcacacaggaaacagctatgaccatgattacgaattctggcacgacaggtttcccgactggaaagcgggcagtgagcgcaacgcaattaatgtgagttagctcactcattaggcaccccaggctttacactttatgcttccggctcgtatgttgtgtggaattgtgagcggataacaatttcacacaggaaacagctatgaccatgattacgccaagcttgcatgcctgcaggtcaacatggtggagcacgacactctcgtctactccaagaatatcaaagatacagtctcagaagaccagagggctattgagacttttcaacaaagggtaatatcgggaaacctcctcggattccattgcccagctatctgtcacttcatcgaaaggacagtagaaaaggaagatggcttctacaaatgccatcattgcgataaaggaaaggctatcgttcaagatgcctctaccgacagtggtcccaaagatggacccccacccacgaggaacatcgtggaaaaagaagacgttccaaccacgtcttcaaagcaagtggattgatgtgatggtcaacatggtggagcacgacactctcgtctactccaagaatatcaaagatacagtctcagaagaccagagggctattgagacttttcaacaaagggtaatatcgggaaacctcctcggattccattgcccagctatctgtcacttcatcgaaaggacagtagaaaaggaagatggcttctacaaatgccatcattgcgataaaggaaaggctatcgttcaagatgcctctaccgacagtggtcccaaagatggacccccacccacgaggaacatcgtggaaaaagaagacgttccaaccacgtcttcaaagcaagtggattgatgtgatatctccactgacgtaagggatgacgcacaatcccactatccttcgcaagacccttcctctatataaggaagttcatttcatttggagaggcctgggtacctctaga

SEQ ID NO: 3 - DNA, 13623 bp, synthetic construct
  source 1..13623: mol_type = other DNA
gtttatttacaagagcgtacggttcaatccctgcctcccctgtaaaattaccctttgaaaacctctcttttctaatcttttctttgtaaattcctatggcgacgtcctcgttcaacattaatgaactggtagcctcccacggcgataaaggactactcgcgaacgccctcgttgataagacagctcatgagcagctcgaggagcaattacagcatcaacgcagaggccgtaaggtctacattcggaacgttctgagtgtaaaggattctgaggtcatccggaatcggtatggaggaaagtacgacctccatcttacccagcaggagtttgctccccacggcctagctggtgccctccgcttgtgtgaaactctcgattgtctagactctttcccttcatcaggtctgcggcaggacctcgttttagacttcggaggaagttgggtcacacattacctccgcggacataacgtacactgttgttccccttgtttgggtattcgcgataaaatgcgccacgcggaacgtttaatgagcatgcgcaagatcatcttgaacgatccacaacagttcgatggtcgacagccggatttttgcactcatcccgctgctgattgcaaagtacaagcccactttgctatatctattcatggaggttatgatatgggctttagaggattatgtgaagcaatgaatgctcacggaaccactattttgaagggaacgatgatgttcgatggtgcgatgatgtttgacgaccaaggcttaatacctgagcttaattgtcagtggaggaagattaggagtgctttctccgaagctgaagacgtcacacctttgtctggtaaaattgattcttcaggattcaccggcgtgcgtaagttcaagactttgatagcttttgattttatcaacgagtctaccatgtcttatgttcatgactggaagaatataaaatcgtttctgacggaccagacgtactcgtataaagggatgacttatggcattgaacgttgtgtcattaatgcgggtatcatgacgtataagattatcggtgtgcctgggatgtgcccacccgaactcattcgacattgtatttggtttccctctattaaggactatgttggtctcaagattcccgcgtcgcaagacttggttaagtggaaaacagtgcgcattttaacgtcaacattgcgtgagactgaagagattgctatgaggtgttataatgataagaaggcgtggatggagcagtttaaggttatcttaggtgttctctccgctaaatcatccaccattgttattaatggtatgtctatgcaatctggcgaacgaatcgatatcaacgattatcattatattggattcgccattcttctccacacaaaaatgaagtatgaacagttagggaagatgtatgatatgtggaatgcttcgagtatctcgaagtggttcgccgcgttgactcgtccgctgcgtgtgttcttctctagcgttgttcacgcactgttcccgactttgagaccccgcgaggagaaagaatttctgattaagctctccacctttgtgactttcaacgaagagtgctcgtttgatggtggagaggaatgggacgtgatatcatctgctgcattcgttgccacgcaggctgttaccgatgggaagattttggccgcgcagaaggccgagaagctcgctgaaaagcttgcgcaacccgtgattgaggtatcggacagtcctgaagcgtcatcttcaacgcttgatgatactgctgatgtttgtggaagggagcaagaagtttcggagcttgactccctgtcagttcagacacgttcccccatcactagaattgctgaaagggctactgctatgttagagtatgccgcttatgagaaacagttgcatgacaccacggtgtccaacctgaaacgcatttggaatatggcgggtggtgatgacaagaaaaattccctcgaaggcaatttgaagtttgtctttgacacgtattttaccgttgatcctatggtgaatgttcatttctccacaggtcggtggatgcgtcctgtgcctgaagggattgcttattctgtcggttataatgaacgcggtctaggtccgaaatccgatggggagctttacattgttaatagtgagtgtgtgatcagtaacagcgagtctttgtctgctgtcacacgctcgttacaagctcccaccggcaccattagtcaagttgatggggtcgctgggtgcgggaaaaccacagcaattaaatcaatttttgagccgtccacggatatgatcgttaccgctaacaagaaatccgcccaagatgtgcgtatggcacttttcaaatcgtcggactccaaagaagcttgcacctttgtccgaacagccgactctgttttgcttaatgaatgtccgaccgtgagtagagttctggttgatgaggtcgtgctactgcactttggtcaattatgtgccgtcatgtctaaattgaaggctgtgagagctatttgtttcggggattcagagcagattgctttttcctctcgagatgcctcgtttgacatgcgtttctccaagatcatccctgatgaaactagtgacgcggacactacgttccgtagcccacaagacgtcgtgccgcttgtgcgtttgatggctacgaaggccctcccgaaaggaacccgctcaaagtatacgaaatgggtttctcaatccaaagtgaagagatctgtcacatctcgggctattgcgagtgtgacgttggttgatttagatgagtctagattttacgtcacgatgacacaagccgataaagcttcactgatttcaagggcgaaagagatgaacttaccgaagactttctggaatgaaaggattaaaaccgtgcatgagtctcaaggtatttctgaggatcacgttactttggtaagattaaagagcacaaagtgtgacctgttcaagaaattttcttactgtcttgtcgctttaactaggcataaggtcaccttccgctacgagtattgtggtgcattgaacggcgatttaattgccgagtgtgttgctcgtgtttagcggtgcccctccttcgggcgggatctgagttggcggtaatctacaaaccgtctgaagtcactaaacgctttgcggtgaacgggttgtccatccagcttacggctaaaatggtcagtcgtggagaaattcacgccagtagacttacaagtctctaaggtgcctttgaaaccatctcctaggtttcttcggaaggacttcggtccgtgtacttctagcacaacgtgctagtttcagggtacgggtgcccccccactttcgtgggggtctctcaaaggagaccaggatccgataccctgtcaccggatgtgttttccggtctgatgagtccgtgaggacgaaacaggactgtcctgcaggagctcgaattcggtacgctgaaatcaccagtctctctctacaaatctatctctctctattttctccataaataatgtgtgagtagtttccgataaggaaattagggttcttatagggtttcgtcatgtgttgagcatataagaaacccttagtatgtatttgtatttgtaaaatacttctatcaataaaatttctaattcctaaaaccaaaatcagtactaaatcagatccccaattcactggccgtcgttttacaacgtcgtgactgggaaaaccctggcgttacccaacttaatcgccttgcagcacatccccctttcgccagtggcactggccgtcgttttacaacgtcgtgactgggaaaaccctggcgttacccaacttaatcgccttgcagcacatccccctttcgccagctggcgtaatagcgaagaggcccgcaccgatcgcccttcccaacagttgcgcagcctgaatggcgaatgctagagcagcttgagcttggatcagattgtcgtttcccgccttcagtttaaactatcagtgtttgacaggatatattggcgggtaaacctaagagaaaagagcgtttattagaataacggatatttaaaagggcgtgaaaaggtttatccgttcgtccatttgtatgtgcatgccaaccacagggttcccctcgggatcaaagtactttgatccaacccctccgctgctatagtgcagtcggcttctgacgttcagtgcagccgtcttctgaaaacgacatgtcgcacaagtcctaagttacgcgacaggctgccgccctgcccttttcctggcgttttcttgtcgcgtgttttagtcgcataaagtagaatacttgcgactagaaccggagacattacgccatgaacaagagcgccgccgctggcctgctgggctatgcccgcgtcagcaccgacgaccaggacttgaccaaccaacgggccgaactgcacgcggccggctgcaccaagctgttttccgagaagatcaccggcaccaggcgcgaccgcccggagctggccaggatgcttgaccacctacgccctggcgacgttgtgacagtgaccaggctagaccgcctggcccgcagcacccgcgacctactggacattgccgagcgcatccaggaggccggcgcgggcctgcgtagcctggcagagccgtgggccgacaccaccacgccggccggccgcatggtgttgaccgtgttcgccggcattgccgagttcgagcgttccctaatcatcgaccgcacccggagcgggcgcgaggccgccaaggcccgaggcgtgaagtttggcccccgccctaccctcaccccggcacagatcgcgcacgcccgcgagctgatcgaccaggaaggccgcaccgtgaaagaggcggctgcactgcttggcgtgcatcgctcgaccctgtaccgcgcacttgagcgcagcgaggaagtgacgcccaccgaggccaggcggcgcggtgccttccgtgaggacgcattgaccgaggccgacgccctggcggccgccgagaatgaacgccaagaggaacaagcatgaaaccgcaccaggacggccaggacgaaccgtttttcattaccgaagagatcgaggcggagatgatcgcggccgggtacgtgttcgagccgcccgcgcacgtctcaaccgtgcggctgcatgaaatcctggccggtttgtctgatgccaagctggcggcctggccggccagcttggccgctgaagaaaccgagcgccgccgtctaaaaaggtgatgtgtatttgagtaaaacagcttgcgtcatgcggtcgctgcgtatatgatgcgatgagtaaataaacaaatacgcaaggggaacgcatgaaggttatcgctgtacttaaccagaaaggcgggtcaggcaagacgaccatcgcaacccatctagcccgcgccctgcaactcgccggggccgatgttctgttagtcgattccgatccccagggcagtgcccgcgattgggcggccgtgcgggaagatcaaccgctaaccgttgtcggcatcgaccgcccgacgattgaccgcgacgtgaaggccatcggccggcgcgacttcgtagtgatcgacggagcgccccaggcggcggacttggctgtgtccgcgatcaaggcagccgacttcgtgctgattccggtgcagccaagcccttacgacatatgggccaccgccgacctggtggagctggttaagcagcgcattgaggtcacggatggaaggctacaagcggcctttgtcgtgtcgcgggcgatcaaaggcacgcgcatcggcggtgaggttgccgaggcgctggccgggtacgagctgcccattcttgagtcccgtatcacgcagcgcgtgagctacccaggcactgccgccgccggcacaaccgttcttgaatcagaacccgagggcgacgctgcccgcgaggtccaggcgctggccgctgaaattaaatcaaaactcatttgagttaatgaggtaaagagaaaatgagcaaaagcacaaacacgctaagtgccggccgtccgagcgcacgcagcagcaaggctgcaacgttggccagcctggcagacacgccagccatgaagcgggtcaactttcagttgccggcggaggatcacaccaagctgaagatgtacgcggtacgccaaggcaagaccattaccgagctgctatctgaatacatcgcgcagctaccagagtaaatgagcaaatgaataaatgagtagatgaattttagcggctaaaggaggcggcatggaaaatcaagaacaaccaggcaccgacgccgtggaatgccccatgtgtggaggaacgggcggttggccaggcgtaagcggctgggttgtctgccggccctgcaatggcactggaacccccaagcccgaggaatcggcgtgacggtcgcaaaccatccggcccggtacaaatcggcgcggcgctgggtgatgacctggtggagaagttgaaggccgcgcaggccgcccagcggcaacgcatcgaggcagaagcacgccccggtgaatcgtggcaagcggccgctgatcgaatccgcaaagaatcccggcaaccgccggcagccggtgcgccgtcgattaggaagccgcccaagggcgacgagcaaccagattttttcgttccgatgctctatgacgtgggcacccgcgatagtcgcagcatcatggacgtggccgttttccgtctgtcgaagcgtgaccgacgagctggcgaggtgatccgctacgagcttccagacgggcacgtagaggtttccgcagggccggccggcatggccagtgtgtgggattacgacctggtactgatggcggtttcccatctaaccgaatccatgaaccgataccgggaagggaagggagacaagcccggccgcgtgttccgtccacacgttgcggacgtactcaagttctgccggcgagccgatggcggaaagcagaaagacgacctggtagaaacctgcattcggttaaacaccacgcacgttgccatgcagcgtacgaagaaggccaagaacggccgcctggtgacggtatccgagggtgaagccttgattagccgctacaagatcgtaaagagcgaaaccgggcggccggagtacatcgagatcgagctagctgattggatgtaccgcgagatcacagaaggcaagaacccggacgtgctgacggttcaccccgattactttttgatcgatcccggcatcggccgttttctctaccgcctggcacgccgcgccgcaggcaaggcagaagccagatggttgttcaagacgatctacgaacgcagtggcagcgccggagagttcaagaagttctgtttcaccgtgcgcaagctgatcgggtcaaatgacctgccggagtacgatttgaaggaggaggcggggcaggctggcccgatcctagtcatgcgctaccgcaacctgatcgagggcgaagcatccgccggttcctaatgtacggagcagatgctagggcaaattgccctagcaggggaaaaaggtcgaaaaggtctctttcctgtggatagcacgtacattgggaacccaaagccgtacattgggaaccggaacccgtacattgggaacccaaagccgtacattgggaaccggtcacacatgtaagtgactgatataaaagagaaaaaaggcgatttttccgcctaaaactctttaaaacttattaaaactcttaaaacccgcctggcctgtgcataactgtctggccagcgcacagccgaagagctgcaaaaagcgcctacccttcggtcgctgcgctccctacgccccgccgcttcgcgtcggcctatcgcggccgctggccgctcaaaaatggctggcctacggccaggcaatctaccagggcgcggacaagccgcgccgtcgccactcgaccgccggcgcccacatcaaggcaccctgcctcgcgcgtttcggtgatgacggtgaaaacctctgacacatgcagctcccggagacggtcacagcttgtctgtaagcggatgccgggagcagacaagcccgtcagggcgcgtcagcgggtgttggcgggtgtcggggcgcagccatgacccagtcacgtagcgatagcggagtgtatactggcttaactatgcggcatcagagcagattgtactgagagtgcaccatatgcggtgtgaaataccgcacagatgcgtaaggagaaaataccgcatcaggcgctcttccgcttcctcgctcactgactcgctgcgctcggtcgttcggctgcggcgagcggtatcagctcactcaaaggcggtaatacggttatccacagaatcaggggataacgcaggaaagaacatgtgagcaaaaggccagcaaaaggccaggaaccgtaaaaaggccgcgttgctggcgtttttccataggctccgcccccctgacgagcatcacaaaaatcgacgctcaagtcagaggtggcgaaacccgacaggactataaagataccaggcgtttccccctggaagctccctcgtgcgctctcctgttccgaccctgccgcttaccggatacctgtccgcctttctcccttcgggaagcgtggcgctttctcatagctcacgctgtaggtatctcagttcggtgtaggtcgttcgctccaagctgggctgtgtgcacgaaccccccgttcagcccgaccgctgcgccttatccggtaactatcgtcttgagtccaacccggtaagacacgacttatcgccactggcagcagccactggtaacaggattagcagagcgaggtatgtaggcggtgctacagagttcttgaagtggtggcctaactacggctacactagaaggacagtatttggtatctgcgctctgctgaagccagttaccttcggaaaaagagttggtagctcttgatccggcaaacaaaccaccgctggtagcggtggtttttttgtttgcaagcagcagattacgcgcagaaaaaaaggatctcaagaagatcctttgatcttttctacggggtctgacgctcagtggaacgaaaactcacgttaagggattttggtcatgcattctaggtactaaaacaattcatccagtaaaatataatattttattttctcccaatcaggcttgatccccagtaagtcaaaaaatagctcgacatactgttcttccccgatatcctccctgatcgaccggacgcagaaggcaatgtcataccacttgtccgccctgccgcttctcccaagatcaataaagccacttactttgccatctttcacaaagatgttgctgtctcccaggtcgccgtgggaaaagacaagttcctcttcgggcttttccgtctttaaaaaatcatacagctcgcgcggatctttaaatggagtgtcttcttcccagttttcgcaatccacatcggccagatcgttattcagtaagtaatccaattcggctaagcggctgtctaagctattcgtatagggacaatccgatatgtcgatggagtgaaagagcctgatgcactccgcatacagctcgataatcttttcagggctttgttcatcttcatactcttccgagcaaaggacgccatcggcctcactcatgagcagattgctccagccatcatgccgttcaaagtgcaggacctttggaacaggcagctttccttccagccatagcatcatgtccttttcccgttccacatcataggtggtccctttataccggctgtccgtcatttttaaatataggttttcattttctcccaccagcttatataccttagcaggagacattccttccgtatcttttacgcagcggtatttttcgatcagttttttcaattccggtgatattctcattttagccatttattatttccttcctcttttctacagtatttaaagataccccaagaagctaattataacaagacgaactccaattcactgttccttgcattctaaaaccttaaataccagaaaacagctttttcaaagttgttttcaaagttggcgtataacatagtatcgacggagccgattttgaaaccgcggtgatcacaggcagcaacgctctgtcatcgttacaatcaacatgctaccctccgcgagatcatccgtgtttcaaacccggcagcttagttgccgttcttccgaatagcatcggtaacatgagcaaagtctgccgccttacaacggctctcccgctgacgccgtcccggactgatgggctgcctgtatcgagtggtgattttgtgccgagctgccggtcggggagctgttggctggctggtggcaggatatattgtggtgtaaacaaattgacgcttagacaacttaataacacattgcggacgtttttaatgtactgaattaacgccgaattaattcgggggatctggattttagtactggattttggttttaggaattagaaattttattgatagaagtattttacaaatacaaatacatactaagggtttcttatatgctcaacacatgagcgaaaccctataggaaccctaattcccttatctgggaactactcacacattattatggagaaactcgagcttgtcgatcgacagatccggtcggcatctactctatttctttgccctcggacgagtgctggggcgtcggtttccactatcggcgagtacttctacacagccatcggtccagacggccgcgcttctgcgggcgatttgtgtacgcccgacagtcccggctccggatcggacgattgcgtcgcatcgaccctgcgcccaagctgcatcatcgaaattgccgtcaaccaagctctgatagagttggtcaagaccaatgcggagcatatacgcccggagtcgtggcgatcctgcaagctccggatgcctccgctcgaagtagcgcgtctgctgctccatacaagccaaccacggcctccagaagaagatgttggcgacctcgtattgggaatccccgaacatcgcctcgctccagtcaatgaccgctgttatgcggccattgtccgtcaggacattgttggagccgaaatccgcgtgcacgaggtgccggacttcggggcagtcctcggcccaaagcatcagctcatcgagagcctgcgcgacggacgcactgacggtgtcgtccatcacagtttgccagtgatacacatggggatcagcaatcgcgcatatgaaatcacgccatgtagtgtattgaccgattccttgcggtccgaatgggccgaacccgctcgtctggctaagatcggccgcagcgatcgcatccatagcctccgcgaccggttgtagaacagcgggcagttcggtttcaggcaggtcttgcaacgtgacaccctgtgcacggcgggagatgcaataggtcaggctctcgctaaactccccaatgtcaagcacttccggaatcgggagcgcggccgatgcaaagtgccgataaacataacgatctttgtagaaaccatcggcgcagctatttacccgcaggacatatccacgccctcctacatcgaagctgaaagcacgagattcttcgccctccgagagctgcatcaggtcggagacgctgtcgaacttttcgatcagaaacttctcgacagacgtcgcggtgagttcaggctttttcatatctcattgccccccgggatctgcgaaagctcgagagagatagatttgtagagagagactggtgatttcagcgtgtcctctccaaatgaaatgaacttccttatatagaggaaggtcttgcgaaggatagtgggattgtgcgtcatcccttacgtcagtggagatatcacatcaatccacttgctttgaagacgtggttggaacgtcttctttttccacgatgctcctcgtgggtgggggtccatctttgggaccactgtcggcagaggcatcttgaacgatagcctttcctttatcgcaatgatggcatttgtaggtgccaccttccttttctactgtccttttgatgaagtgacagatagctgggcaatggaatccgaggaggtttcccgatattaccctttgttgaaaagtctcaatagccctttggtcttctgagactgtatctttgatattcttggagtagacgagagtgtcgtgctccaccatgttatcacatcaatccacttgctttgaagacgtggttggaacgtcttctttttccacgatgctcctcgtgggtgggggtccatctttgggaccactgtcggcagaggcatcttgaacgatagcctttcctttatcgcaatgatggcatttgtaggtgccaccttccttttctactgtccttttgatgaagtgacagatagctgggcaatggaatccgaggaggtttcccgatattaccctttgttgaaaagtctcaatagccctttggtcttctgagactgtatctttgatattcttggagtagacgagagtgtcgtgctccaccatgttggcaagctgctctagccaatacgcaaaccgcctctccccgcgcgttggccgattcattaatgcagctggcacgacaggtttcccgactggaaagcgggcagtgagcgcaacgcaattaatgtgagttagctcactcattaggcaccccaggctttacactttatgcttccggctcgtatgttgtgtggaattgtgagcggataacaatttcacacaggaaacagctatgaccatgattacgaattctggcacgacaggtttcccgactggaaagcgggcagtgagcgcaacgcaattaatgtgagttagctcactcattaggcaccccaggctttacactttatgcttccggctcgtatgttgtgtggaattgtgagcggataacaatttcacacaggaaacagctatgaccatgattacgccaagcttgcatgcctgcaggtcaacatggtggagcacgacactctcgtctactccaagaatatcaaagatacagtctcagaagaccagagggctattgagacttttcaacaaagggtaatatcgggaaacctcctcggattccattgcccagctatctgtcacttcatcgaaaggacagtagaaaaggaagatggcttctacaaatgccatcattgcgataaaggaaaggctatcgttcaagatgcctctaccgacagtggtcccaaagatggacccccacccacgaggaacatcgtggaaaaagaagacgttccaaccacgtcttcaaagcaagtggattgatgtgatggtcaacatggtggagcacgacactctcgtctactccaagaatatcaaagatacagtctcagaagaccagagggctattgagacttttcaacaaagggtaatatcgggaaacctcctcggattccattgcccagctatctgtcacttcatcgaaaggacagtagaaaaggaagatggcttctacaaatgccatcattgcgataaaggaaaggctatcgttcaagatgcctctaccgacagtggtcccaaagatggacccccacccacgaggaacatcgtggaaaaagaagacgttccaaccacgtcttcaaagcaagtggattgatgtgatatctccactgacgtaagggatgacgcacaatcccactatccttcgcaagacccttcctctatataaggaagttcatttcatttggagaggcctgggtacc

SEQ ID NO: 4 - DNA, 13316 bp, synthetic construct
  source 1..13316: mol_type = other DNA
gtttatttacaagagcgtacggttcaacccctgcctcccctgtaaaattccctagactttctagtttctttctttcctatggctttccctgcccccgctttctcattggccaatcttttgaatggtacttacggtgtcgacactcccgaggaagtggaacgtgtgcgatctgagcaacacgaagaggctgctgcggcttgtcgtaattacaagcctttacccgctgtggatgtcagcgagagtgtcacagaggatgcgcattccctccgaactccagacggagctccctttgaagaggtgtctgttgagctcgttacttttggtgctgaagattaccttggaaaatctgatgatgagctccttgtcgcttttgagacgatggtcaaacccatgtgtatcggacagttatggtgccctgcgtttaataaatgttcttttatttccagcattgctatggctagagctttgctgttggtacctagcacatccaaccgaaccatgaagtgttttgaagacctggtcgcggctatttacactaaatccgatttctattacgatgatgagtgtgaagctgacgacattcagataaatgtctcgtctcgcgatgtacccggttattctttcgaaccgtggtcccgaacatctggatttgaaccaccgcctatctgtgaggcgtgtgacatgatcatgtaccagtgcccgtgttttgattttaatgctttaaagaaatcgtgcgctgagaggactttcgctgatgactatgttattgaaggtttagatggtgttgttgacaatgcaactttgttgtctaatttaggcccatttttggtgcctgtgaagtgccaatacgagaaatgtccaacacccaccgtcgcgactcctccgagtttaaatcgtgctactgatcgtgttgatatcaatttagttcaatccatttgtgattccactctgcccacgcatagcaactacgatgactcttttcatcaagtgttcgtcgaaagcgctgattattctattgatctggatcatgttagacttcggcaatctgatctcattgcaaaaattccagaatcagggcatatgataccggttttaaataccgggagtggtcacaagagagtaggtacgacgaaggaggtccttacagcaatcaagaaacgtaatgctgacgttccagagctaggtgattccgttaatctgtccaggttgagtaaggctgtggctgagagatttttcatctcgtacattaatggcaactctttagccaccagcaactttgttaacgtcgttagcaatttccacgattacatggaaaaatggaagtcttcaggtctctcgtatgacgatcttccagatctgcatgctgagaatttgcagttttatgatcacatgataaaatctgatgtgaagcctgtcgttagcgacacattgaacattgacagaccggttccagctactataacgtatcacaagaaaggtataacctcccagttctcaccgttattcacagctctatttgagcgtttccagagatgccttcgagaacgtattattcttcctgttggaaagatttcatcccttgagatgtcaggatttgatgttaagaacaaacattgtctcgagatcgatttgtccaaattcgacaagtctcaaggtgaattccatttgatgattcaggaacacattttgaatggtctagggtgcccagctccgataactaagtggtggtgtgatttccacagattctcttacattagagaccgtagagctggtgttggtatgcctatcagtttccagagacgaactggtgatgcatttacctacttcggtaacaccatcgtcaccatggctgaatttgcatggtgttacgacaccgaccaattcgaaaagcttttattctcaggcgatgattctctaggattttcagtgcttccccctgttggcgatccgagtaagttcacaactcttttcaacatggaagctaaggtgatggagccagcagtaccatacatttgttcgaagtttctactctctgatgagttcggtaataccttttccgttccagatccattgcgcgaggttcagcggttaggaactaagaaaatcccctattccgacaatgacgaattcctgtttgctcacttcatgagctttgttgatcgattgaagtttttggaccgaatgactcagtcttgcatcgatcagctttcactcttctttgagttgaaatacaggaagtccggggcggaggctgccttgatgttaggcgcctttaagaaatataccgctaattttcagtcctacaaagaactctatttttcagatcgtcgtcagtgcgaattgatcaattcgtttagttgtgtagagttgaggattgagcgttcgagtttcattaagcagcgaaagaagaaagatggaattgaacgaaggcgcaatgacaaacgtcgaactccaactagcccgcatggtggaggcgaagagacagagacgaaggtctcacaagaagaatcgacgggaacgatgttacaaaagtcccagcgagagagcacgttcaaatctcagactgttccgcttcctaccgttctatcaagtagatggttcggaactgatagagatgtaccgccacgtgaacgtggcggaattgtccgagtctgaggctccttgttttacgttaccagcggaagatgaccatgattttgacgatacagattggttcgctggtaacgagtgggcggaaggtgcgttctgaacccctccttcctttctccctccagttttctgaggcgggagctgagttggcagtattgctacaaactgtctgaagtcactaaacgttttacggtgaacgggttgtccatccagctaacggctaaaatggtcagtcgcggagaaatccacgccggagatttacaagtctctgaggcacctttgaaaccatctcctaggtttcttcggaaggacttcggtccgtgtacttctagcacaacgtgctagtttcagggtacgggtgccccccacttttgtggggcttcctgaaggagaccaggatccgataccctgtcaccggatgtgttttccggtctgatgagtccgtgaggacgaaacaggactgtcctgcaggagctcgaattcggtacgctgaaatcaccagtctctctctacaaatctatctctctctattttctccataaataatgtgtgagtagtttccgataaggaaattagggttcttatagggtttcgtcatgtgttgagcatataagaaacccttagtatgtatttgtatttgtaaaatacttctatcaataaaatttctaattcctaaaaccaaaatcagtactaaatcagatccccaattcactggccgtcgttttacaacgtcgtgactgggaaaaccctggcgttacccaacttaatcgccttgcagcacatccccctttcgccagtggcactggccgtcgttttacaacgtcgtgactgggaaaaccctggcgttacccaacttaatcgccttgcagcacatccccctttcgccagctggcgtaatagcgaagaggcccgcaccgatcgcccttcccaacagttgcgcagcctgaatggcgaatgctagagcagcttgagcttggatcagattgtcgtttcccgccttcagtttaaactatcagtgtttgacaggatatattggcgggtaaacctaagagaaaagagcgtttattagaataacggatatttaaaagggcgtgaaaaggtttatccgttcgtccatttgtatgtgcatgccaaccacagggttcccctcgggatcaaagtactttgatccaacccctccgctgctatagtgcagtcggcttctgacgttcagtgcagccgtcttctgaaaacgacatgtcgcacaagtcctaagttacgcgacaggctgccgccctgcccttttcctggcgttttcttgtcgcgtgttttagtcgcataaagtagaatacttgcgactagaaccggagacattacgccatgaacaagagcgccgccgctggcctgctgggctatgcccgcgtcagcaccgacgaccaggacttgaccaaccaacgggccgaactgcacgcggccggctgcaccaagctgttttccgagaagatcaccggcaccaggcgcgaccgcccggagctggccaggatgcttgaccacctacgccctggcgacgttgtgacagtgaccaggctagaccgcctggcccgcagcacccgcgacctactggacattgccgagcgcatccaggaggccggcgcgggcctgcgtagcctggcagagccgtgggccgacaccaccacgccggccggccgcatggtgttgaccgtgttcgccggcattgccgagttcgagcgttccctaatcatcgaccgcacccggagcgggcgcgaggccgccaaggcccgaggcgtgaagtttggcccccgccctaccctcaccccggcacagatcgcgcacgcccgcgagctgatcgaccaggaaggccgcaccgtgaaagaggcggctgcactgcttggcgtgcatcgctcgaccctgtaccgcgcacttgagcgcagcgaggaagtgacgcccaccgaggccaggcggcgcggtgccttccgtgaggacgcattgaccgaggccgacgccctggcggccgccgagaatgaacgccaagaggaacaagcatgaaaccgcaccaggacggccaggacgaaccgtttttcattaccgaagagatcgaggcggagatgatcgcggccgggtacgtgttcgagccgcccgcgcacgtctcaaccgtgcggctgcatgaaatcctggccggtttgtctgatgccaagctggcggcctggccggccagcttggccgctgaagaaaccgagcgccgccgtctaaaaaggtgatgtgtatttgagtaaaacagcttgcgtcatgcggtcgctgcgtatatgatgcgatgagtaaataaacaaatacgcaaggggaacgcatgaaggttatcgctgtacttaaccagaaaggcgggtcaggcaagacgaccatcgcaacccatctagcccgcgccctgcaactcgccggggccgatgttctgttagtcgattccgatccccagggcagtgcccgcgattgggcggccgtgcgggaagatcaaccgctaaccgttgtcggcatcgaccgcccgacgattgaccgcgacgtgaaggccatcggccggcgcgacttcgtagtgatcgacggagcgccccaggcggcggacttggctgtgtccgcgatcaaggcagccgacttcgtgctgattccggtgcagccaagcccttacgacatatgggccaccgccgacctggtggagctggttaagcagcgcattgaggtcacggatggaaggctacaagcggcctttgtcgtgtcgcgggcgatcaaaggcacgcgcatcggcggtgaggttgccgaggcgctggccgggtacgagctgcccattcttgagtcccgtatcacgcagcgcgtgagctacccaggcactgccgccgccggcacaaccgttcttgaatcagaacccgagggcgacgctgcccgcgaggtccaggcgctggccgctgaaattaaatcaaaactcatttgagttaatgaggtaaagagaaaatgagcaaaagcacaaacacgctaagtgccggccgtccgagcgcacgcagcagcaaggctgcaacgttggccagcctggcagacacgccagccatgaagcgggtcaactttcagttgccggcggaggatcacaccaagctgaagatgtacgcggtacgccaaggcaagaccattaccgagctgctatctgaatacatcgcgcagctaccagagtaaatgagcaaatgaataaatgagtagatgaattttagcggctaaaggaggcggcatggaaaatcaagaacaaccaggcaccgacgccgtggaatgccccatgtgtggaggaacgggcggttggccaggcgtaagcggctgggttgtctgccggccctgcaatggcactggaacccccaagcccgaggaatcggcgtgacggtcgcaaaccatccggcccggtacaaatcggcgcggcgctgggtgatgacctggtggagaagttgaaggccgcgcaggccgcccagcggcaacgcatcgaggcagaagcacgccccggtgaatcgtggcaagcggccgctgatcgaatccgcaaagaatcccggcaaccgccggcagccggtgcgccgtcgattaggaagccgcccaagggcgacgagcaaccagattttttcgttccgatgctctatgacgtgggcacccgcgatagtcgcagcatcatggacgtggccgttttccgtctgtcgaagcgtgaccgacgagctggcgaggtgatccgctacgagcttccagacgggcacgtagaggtttccgcagggccggccggcatggccagtgtgtgggattacgacctggtactgatggcggtttcccatctaaccgaatccatgaaccgataccgggaagggaagggagacaagcccggccgcgtgttccgtccacacgttgcggacgtactcaagttctgccggcgagccgatggcggaaagcagaaagacgacctggtagaaacctgcattcggttaaacaccacgcacgttgccatgcagcgtacgaagaaggccaagaacggccgcctggtgacggtatccgagggtgaagccttgattagccgctacaagatcgtaaagagcgaaaccgggcggccggagtacatcgagatcgagctagctgattggatgtaccgcgagatcacagaaggcaagaacccggacgtgctgacggttcaccccgattactttttgatcgatcccggcatcggccgttttctctaccgcctggcacgccgcgccgcaggcaaggcagaagccagatggttgttcaagacgatctacgaacgcagtggcagcgccggagagttcaagaagttctgtttcaccgtgcgcaagctgatcgggtcaaatgacctgccggagtacgatttgaaggaggaggcggggcaggctggcccgatcctagtcatgcgctaccgcaacctgatcgagggcgaagcatccgccggttcctaatgtacggagcagatgctagggcaaattgccctagcaggggaaaaaggtcgaaaaggtctctttcctgtggatagcacgtacattgggaacccaaagccgtacattgggaaccggaacccgtacattgggaacccaaagccgtacattgggaaccggtcacacatgtaagtgactgatataaaagagaaaaaaggcgatttttccgcctaaaactctttaaaacttattaaaactcttaaaacccgcctggcctgtgcataactgtctggccagcgcacagccgaagagctgcaaaaagcgcctacccttcggtcgctgcgctccctacgccccgccgcttcgcgtcggcctatcgcggccgctggccgctcaaaaatggctggcctacggccaggcaatctaccagggcgcggacaagccgcgccgtcgccactcgaccgccggcgcccacatcaaggcaccctgcctcgcgcgtttcggtgatgacggtgaaaacctctgacacatgcagctcccggagacggtcacagcttgtctgtaagcggatgccgggagcagacaagcccgtcagggcgcgtcagcgggtgttggcgggtgtcggggcgcagccatgacccagtcacgtagcgatagcggagtgtatactggcttaactatgcggcatcagagcagattgtactgagagtgcaccatatgcggtgtgaaataccgcacagatgcgtaaggagaaaataccgcatcaggcgctcttccgcttcctcgctcactgactcgctgcgctcggtcgttcggctgcggcgagcggtatcagctcactcaaaggcggtaatacggttatccacagaatcaggggataacgcaggaaagaacatgtgagcaaaaggccagcaaaaggccaggaaccgtaaaaaggccgcgttgctggcgtttttccataggctccgcccccctgacgagcatcacaaaaatcgacgctcaagtcagaggtggcgaaacccgacaggactataaagataccaggcgtttccccctggaagctccctcgtgcgctctcctgttccgaccctgccgcttaccggatacctgtccgcctttctcccttcgggaagcgtggcgctttctcatagctcacgctgtaggtatctcagttcggtgtaggtcgttcgctccaagctgggctgtgtgcacgaaccccccgttcagcccgaccgctgcgccttatccggtaactatcgtcttgagtccaacccggtaagacacgacttatcgccactggcagcagccactggtaacaggattagcagagcgaggtatgtaggcggtgctacagagttcttgaagtggtggcctaactacggctacactagaaggacagtatttggtatctgcgctctgctgaagccagttaccttcggaaaaagagttggtagctcttgatccggcaaacaaaccaccgctggtagcggtggtttttttgtttgcaagcagcagattacgcgcagaaaaaaaggatctcaagaagatcctttgatcttttctacggggtctgacgctcagtggaacgaaaactcacgttaagggattttggtcatgcattctaggtactaaaacaattcatccagtaaaatataatattttattttctcccaatcaggcttgatccccagtaagtcaaaaaatagctcgacatactgttcttccccgatatcctccctgatcgaccggacgcagaaggcaatgtcataccacttgtccgccctgccgcttctcccaagatcaataaagccacttactttgccatctttcacaaagatgttgctgtctcccaggtcgccgtgggaaaagacaagttcctcttcgggcttttccgtctttaaaaaatcatacagctcgcgcggatctttaaatggagtgtcttcttcccagttttcgcaatccacatcggccagatcgttattcagtaagtaatccaattcggctaagcggctgtctaagctattcgtatagggacaatccgatatgtcgatggagtgaaagagcctgatgcactccgcatacagctcgataatcttttcagggctttgttcatcttcatactcttccgagcaaaggacgccatcggcctcactcatgagcagattgctccagccatcatgccgttcaaagtgcaggacctttggaacaggcagctttccttccagccatagcatcatgtccttttcccgttccacatcataggtggtccctttataccggctgtccgtcatttttaaatataggttttcattttctcccaccagcttatataccttagcaggagacattccttccgtatcttttacgcagcggtatttttcgatcagttttttcaattccggtgatattctcattttagccatttattatttccttcctcttttctacagtatttaaagataccccaagaagctaattataacaagacgaactccaattcactgttccttgcattctaaaaccttaaataccagaaaacagctttttcaaagttgttttcaaagttggcgtataacatagtatcgacggagccgattttgaaaccgcggtgatcacaggcagcaacgctctgtcatcgttacaatcaacatgctaccctccgcgagatcatccgtgtttcaaacccggcagcttagttgccgttcttccgaatagcatcggtaacatgagcaaagtctgccgccttacaacggctctcccgctgacgccgtcccggactgatgggctgcctgtatcgagtggtgattttgtgccgagctgccggtcggggagctgttggctggctggtggcaggatatattgtggtgtaaacaaattgacgcttagacaacttaataacacattgcggacgtttttaatgtactgaattaacgccgaattaattcgggggatctggattttagtactggattttggttttaggaattagaaattttattgatagaagtattttacaaatacaaatacatactaagggtttcttatatgctcaacacatgagcgaaaccctataggaaccctaattcccttatctgggaactactcacacattattatggagaaactcgagcttgtcgatcgacagatccggtcggcatctactctatttctttgccctcggacgagtgctggggcgtcggtttccactatcggcgagtacttctacacagccatcggtccagacggccgcgcttctgcgggcgatttgtgtacgcccgacagtcccggctccggatcggacgattgcgtcgcatcgaccctgcgcccaagctgcatcatcgaaattgccgtcaaccaagctctgatagagttggtcaagaccaatgcggagcatatacgcccggagtcgtggcgatcctgcaagctccggatgcctccgctcgaagtagcgcgtctgctgctccatacaagccaaccacggcctccagaagaagatgttggcgacctcgtattgggaatccccgaacatcgcctcgctccagtcaatgaccgctgttatgcggccattgtccgtcaggacattgttggagccgaaatccgcgtgcacgaggtgccggacttcggggcagtcctcggcccaaagcatcagctcatcgagagcctgcgcgacggacgcactgacggtgtcgtccatcacagtttgccagtgatacacatggggatcagcaatcgcgcatatgaaatcacgccatgtagtgtattgaccgattccttgcggtccgaatgggccgaacccgctcgtctggctaagatcggccgcagcgatcgcatccatagcctccgcgaccggttgtagaacagcgggcagttcggtttcaggcaggtcttgcaacgtgacaccctgtgcacggcgggagatgcaataggtcaggctctcgctaaactccccaatgtcaagcacttccggaatcgggagcgcggccgatgcaaagtgccgataaacataacgatctttgtagaaaccatcggcgcagctatttacccgcaggacatatccacgccctcctacatcgaagctgaaagcacgagattcttcgccctccgagagctgcatcaggtcggagacgctgtcgaacttttcgatcagaaacttctcgacagacgtcgcggtgagttcaggctttttcatatctcattgccccccgggatctgcgaaagctcgagagagatagatttgtagagagagactggtgatttcagcgtgtcctctccaaatgaaatgaacttccttatatagaggaaggtcttgcgaaggatagtgggattgtgcgtcatcccttacgtcagtggagatatcacatcaatccacttgctttgaagacgtggttggaacgtcttctttttccacgatgctcctcgtgggtgggggtccatctttgggaccactgtcggcagaggcatcttgaacgatagcctttcctttatcgcaatgatggcatttgtaggtgccaccttccttttctactgtccttttgatgaagtgacagatagctgggcaatggaatccgaggaggtttcccgatattaccctttgttgaaaagtctcaatagccctttggtcttctgagactgtatctttgatattcttggagtagacgagagtgtcgtgctccaccatgttatcacatcaatccacttgctttgaagacgtggttggaacgtcttctttttccacgatgctcctcgtgggtgggggtccatctttgggaccactgtcggcagaggcatcttgaacgatagcctttcctttatcgcaatgatggcatttgtaggtgccaccttccttttctactgtccttttgatgaagtgacagatagctgggcaatggaatccgaggaggtttcccgatattaccctttgttgaaaagtctcaatagccctttggtcttctgagactgtatctttgatattcttggagtagacgagagtgtcgtgctccaccatgttggcaagctgctctagccaatacgcaaaccgcctctccccgcgcgttggccgattcattaatgcagctggcacgacaggtttcccgactggaaagcgggcagtgagcgcaacgcaattaatgtgagttagctcactcattaggcaccccaggctttacactttatgcttccggctcgtatgttgtgtggaattgtgagcggataacaatttcacacaggaaacagctatgaccatgattacgaattctggcacgacaggtttcccgactggaaagcgggcagtgagcgcaacgcaattaatgtgagttagctcactcattaggcaccccaggctttacactttatgcttccggctcgtatgttgtgtggaattgtgagcggataacaatttcacacaggaaacagctatgaccatgattacgccaagcttgcatgcctgcaggtcaacatggtggagcacgacactctcgtctactccaagaatatcaaagatacagtctcagaagaccagagggctattgagacttttcaacaaagggtaatatcgggaaacctcctcggattccattgcccagctatctgtcacttcatcgaaaggacagtagaaaaggaagatggcttctacaaatgccatcattgcgataaaggaaaggctatcgttcaagatgcctctaccgacagtggtcccaaagatggacccccacccacgaggaacatcgtggaaaaagaagacgttccaaccacgtcttcaaagcaagtggattgatgtgatggtcaacatggtggagcacgacactctcgtctactccaagaatatcaaagatacagtctcagaagaccagagggctattgagacttttcaacaaagggtaatatcgggaaacctcctcggattccattgcccagctatctgtcacttcatcgaaaggacagtagaaaaggaagatggcttctacaaatgccatcattgcgataaaggaaaggctatcgttcaagatgcctctaccgacagtggtcccaaagatggacccccacccacgaggaacatcgtggaaaaagaagacgttccaaccacgtcttcaaagcaagtggattgatgtgatatctccactgacgtaagggatgacgcacaatcccactatccttcgcaagacccttcctctatataaggaagttcatttcatttggagaggcctgggtacctctaga

SEQ ID NO: 5 - DNA, 12484 bp, synthetic construct
  source 1..12484: mol_type = other DNA
gtaatcttaccactgtgtgtgtgtgtgtgtgtgtgtcgcgtcgtgtcgtgtcgtgttgtccgcacatttgagtcgtgctgtccgcaccttttctttcagtgtgttagaatacccgaggcatggctttccaaggtaccagcaggactttaactcaacagtcctcagcggctacgtctgacgaacttcaaaagatattatttagccctgaagccattaagaaaatggctgctgagtgtgacctaggccggcatcattggatgcgagctgataatgctatttcagtccggcccctcgttcccgaagtaacccacggtcgcattgtttctttctttaagtctgggtatgatgctggtgaattgtgctctaaaggatacatgagcgtccctcaagtgttgtgtgctgttactcgaacagtttccactgatgctgaagggtctctgagaatttacctagctgacttaggcgacaaggaattatctcccatagataagcaatgtgtcacattacataaccatgatctccccgctttagtgtctttccaaccgacgtatgattgtcctatggagacagttgggaatcggaagcggtgttttgctgtcgttattgagagacatggttacgttgggtataccggcaccacagctagcgtgtgtagtaattggcaagcacggttttcttctaagaataacaactacactcatatcgcagctgggaagactctagtactgccattcaatagattagctgagcaaacgaaaccgtcagccgtcgctcgcctattgaagtcgcaattgaataacatagaagcttcgcaatacgttttgacggattcgaagatcaatcagaatgcgcgcagtgagtccgaggaattaaatgttgagagccctcccgccgcaatcgggagttcttccgcgtcccgcttcgaaaccttcagaccgcaggtggttaacggtctttagattttcgtcgcgtattagtatataagtatgtgtgagtctgtacataatactatatctatagtgtcctgtgtgagttgatacagtagacaactgtgacgcgatgtcgtgttgagaagggaacacatctggttctagtaagccacatcattagttttgaggttcaattcctcttactccctgttgtgccccttactttttcatggatgcttctccacgaaattgcgtttcgtctactagatcaaggagtgtttgtgttgtgattttctctttgtgttgtagatatttgagtcgagtcatggacaaatctgaatcaaccagtgctggtcgtaaccgtcggcgtcgtccgcgtcgtggttcccgctccgccccctcctccgcggatgctaactttagagtcttgtcgcagcaactttcgcgacttaacaagacgttagcaactggtcgtccaactattaaccacccaaccttcgtgggtagtgagcgttgtaaacctggatacacgttcacttcgattaccctgaagccaccgaaaatagacaaagggtcttattatggtagaaggttggttcttcctgattcagtcacagagttcgataagaagcttgtttcgcgtattcaaattcgagttaatcctttgccgaaatttgattctaccgtgtgggtgacagtccgtaaagttcctgcctcctcggacttatccgttaccgccatctctgctatgttcgcggacggggcctcaccggtactggtttatcagtatgcagcatctggagtccaagccaacaataaattgttgtatgatctttcggcgatgcgcgctgatattggtgacatgagaaagtacgccgtgctcgtgtattcaaaagacgatgcgctcgagacggacgaattggtacttcatgtcgacattgagcaccaacgcattcctacatctggggtgctcccagtttgaacctgtgttttccagaaccctccctccgattctgtggcgggagctgagttggtagtgttgctataaactacctgaagtcactaaacgctatgcggtgaacgggttgtccatccagcttacggctaaaatggtcagtcgtggagaaatccacgccagtagacttacaagtctctgaggtgcctttgaaaccatctcctaggtttcttcggaaggacttcggtccgtgtacttctagcacaagatgctagtttagagtacgggcatcccccattttttttaatggggtctctcaaaggagaccaggatccgataccctgtcaccggatgtgttttccggtctgatgagtccgtgaggacgaaacaggactgtcctgcaggagctcgaattcggtacgctgaaatcaccagtctctctctacaaatctatctctctctattttctccataaataatgtgtgagtagtttccgataaggaaattagggttcttatagggtttcgtcatgtgttgagcatataagaaacccttagtatgtatttgtatttgtaaaatacttctatcaataaaatttctaattcctaaaaccaaaatcagtactaaatcagatccccaattcactggccgtcgttttacaacgtcgtgactgggaaaaccctggcgttacccaacttaatcgccttgcagcacatccccctttcgccagtggcactggccgtcgttttacaacgtcgtgactgggaaaaccctggcgttacccaacttaatcgccttgcagcacatccccctttcgccagctggcgtaatagcgaagaggcccgcaccgatcgcccttcccaacagttgcgcagcctgaatggcgaatgctagagcagcttgagcttggatcagattgtcgtttcccgccttcagtttaaactatcagtgtttgacaggatatattggcgggtaaacctaagagaaaagagcgtttattagaataacggatatttaaaagggcgtgaaaaggtttatccgttcgtccatttgtatgtgcatgccaaccacagggttcccctcgggatcaaagtactttgatccaacccctccgctgctatagtgcagtcggcttctgacgttcagtgcagccgtcttctgaaaacgacatgtcgcacaagtcctaagttacgcgacaggctgccgccctgcccttttcctggcgttttcttgtcgcgtgttttagtcgcataaagtagaatacttgcgactagaaccggagacattacgccatgaacaagagcgccgccgctggcctgctgggctatgcccgcgtcagcaccgacgaccaggacttgaccaaccaacgggccgaactgcacgcggccggctgcaccaagctgttttccgagaagatcaccggcaccaggcgcgaccgcccggagctggccaggatgcttgaccacctacgccctggcgacgttgtgacagtgaccaggctagaccgcctggcccgcagcacccgcgacctactggacattgccgagcgcatccaggaggccggcgcgggcctgcgtagcctggcagagccgtgggccgacaccaccacgccggccggccgcatggtgttgaccgtgttcgccggcattgccgagttcgagcgttccctaatcatcgaccgcacccggagcgggcgcgaggccgccaaggcccgaggcgtgaagtttggcccccgccctaccctcaccccggcacagatcgcgcacgcccgcgagctgatcgaccaggaaggccgcaccgtgaaagaggcggctgcactgcttggcgtgcatcgctcgaccctgtaccgcgcacttgagcgcagcgaggaagtgacgcccaccgaggccaggcggcgcggtgccttccgtgaggacgcattgaccgaggccgacgccctggcggccgccgagaatgaacgccaagaggaacaagcatgaaaccgcaccaggacggccaggacgaaccgtttttcattaccgaagagatcgaggcggagatgatcgcggccgggtacgtgttcgagccgcccgcgcacgtctcaaccgtgcggctgcatgaaatcctggccggtttgtctgatgccaagctggcggcctggccggccagcttggccgctgaagaaaccgagcgccgccgtctaaaaaggtgatgtgtatttgagtaaaacagcttgcgtcatgcggtcgctgcgtatatgatgcgatgagtaaataaacaaatacgcaaggggaacgcatgaaggttatcgctgtacttaaccagaaaggcgggtcaggcaagacgaccatcgcaacccatctagcccgcgccctgcaactcgccggggccgatgttctgttagtcgattccgatccccagggcagtgcccgcgattgggcggccgtgcgggaagatcaaccgctaaccgttgtcggcatcgaccgcccgacgattgaccgcgacgtgaaggccatcggccggcgcgacttcgtagtgatcgacggagcgccccaggcggcggacttggctgtgtccgcgatcaaggcagccgacttcgtgctgattccggtgcagccaagcccttacgacatatgggccaccgccgacctggtggagctggttaagcagcgcattgaggtcacggatggaaggctacaagcggcctttgtcgtgtcgcgggcgatcaaaggcacgcgcatcggcggtgaggttgccgaggcgctggccgggtacgagctgcccattcttgagtcccgtatcacgcagcgcgtgagctacccaggcactgccgccgccggcacaaccgttcttgaatcagaacccgagggcgacgctgcccgcgaggtccaggcgctggccgctgaaattaaatcaaaactcatttgagttaatgaggtaaagagaaaatgagcaaaagcacaaacacgctaagtgccggccgtccgagcgcacgcagcagcaaggctgcaacgttggccagcctggcagacacgccagccatgaagcgggtcaactttcagttgccggcggaggatcacaccaagctgaagatgtacgcggtacgccaaggcaagaccattaccgagctgctatctgaatacatcgcgcagctaccagagtaaatgagcaaatgaataaatgagtagatgaattttagcggctaaaggaggcggcatggaaaatcaagaacaaccaggcaccgacgccgtggaatgccccatgtgtggaggaacgggcggttggccaggcgtaagcggctgggttgtctgccggccctgcaatggcactggaacccccaagcccgaggaatcggcgtgacggtcgcaaaccatccggcccggtacaaatcggcgcggcgctgggtgatgacctggtggagaagttgaaggccgcgcaggccgcccagcggcaacgcatcgaggcagaagcacgccccggtgaatcgtggcaagcggccgctgatcgaatccgcaaagaatcccggcaaccgccggcagccggtgcgccgtcgattaggaagccgcccaagggcgacgagcaaccagattttttcgttccgatgctctatgacgtgggcacccgcgatagtcgcagcatcatggacgtggccgttttccgtctgtcgaagcgtgaccgacgagctggcgaggtgatccgctacgagcttccagacgggcacgtagaggtttccgcagggccggccggcatggccagtgtgtgggattacgacctggtactgatggcggtttcccatctaaccgaatccatgaaccgataccgggaagggaagggagacaagcccggccgcgtgttccgtccacacgttgcggacgtactcaagttctgccggcgagccgatggcggaaagcagaaagacgacctggtagaaacctgcattcggttaaacaccacgcacgttgccatgcagcgtacgaagaaggccaagaacggccgcctggtgacggtatccgagggtgaagccttgattagccgctacaagatcgtaaagagcgaaaccgggcggccggagtacatcgagatcgagctagctgattggatgtaccgcgagatcacagaaggcaagaacccggacgtgctgacggttcaccccgattactttttgatcgatcccggcatcggccgttttctctaccgcctggcacgccgcgccgcaggcaaggcagaagccagatggttgttcaagacgatctacgaacgcagtggcagcgccggagagttcaagaagttctgtttcaccgtgcgcaagctgatcgggtcaaatgacctgccggagtacgatttgaaggaggaggcggggcaggctggcccgatcctagtcatgcgctaccgcaacctgatcgagggcgaagcatccgccggttcctaatgtacggagcagatgctagggcaaattgccctagcaggggaaaaaggtcgaaaaggtctctttcctgtggatagcacgtacattgggaacccaaagccgtacattgggaaccggaacccgtacattgggaacccaaagccgtacattgggaaccggtcacacatgtaagtgactgatataaaagagaaaaaaggcgatttttccgcctaaaactctttaaaacttattaaaactcttaaaacccgcctggcctgtgcataactgtctggccagcgcacagccgaagagctgcaaaaagcgcctacccttcggtcgctgcgctccctacgccccgccgcttcgcgtcggcctatcgcggccgctggccgctcaaaaatggctggcctacggccaggcaatctaccagggcgcggacaagccgcgccgtcgccactcgaccgccggcgcccacatcaaggcaccctgcctcgcgcgtttcggtgatgacggtgaaaacctctgacacatgcagctcccggagacggtcacagcttgtctgtaagcggatgccgggagcagacaagcccgtcagggcgcgtcagcgggtgttggcgggtgtcggggcgcagccatgacccagtcacgtagcgatagcggagtgtatactggcttaactatgcggcatcagagcagattgtactgagagtgcaccatatgcggtgtgaaataccgcacagatgcgtaaggagaaaataccgcatcaggcgctcttccgcttcctcgctcactgactcgctgcgctcggtcgttcggctgcggcgagcggtatcagctcactcaaaggcggtaatacggttatccacagaatcaggggataacgcaggaaagaacatgtgagcaaaaggccagcaaaaggccaggaaccgtaaaaaggccgcgttgctggcgtttttccataggctccgcccccctgacgagcatcacaaaaatcgacgctcaagtcagaggtggcgaaacccgacaggactataaagataccaggcgtttccccctggaagctccctcgtgcgctctcctgttccgaccctgccgcttaccggatacctgtccgcctttctcccttcgggaagcgtggcgctttctcatagctcacgctgtaggtatctcagttcggtgtaggtcgttcgctccaagctgggctgtgtgcacgaaccccccgttcagcccgaccgctgcgccttatccggtaactatcgtcttgagtccaacccggtaagacacgacttatcgccactggcagcagccactggtaacaggattagcagagcgaggtatgtaggcggtgctacagagttcttgaagtggtggcctaactacggctacactagaaggacagtatttggtatctgcgctctgctgaagccagttaccttcggaaaaagagttggtagctcttgatccggcaaacaaaccaccgctggtagcggtggtttttttgtttgcaagcagcagattacgcgcagaaaaaaaggatctcaagaagatcctttgatcttttctacggggtctgacgctcagtggaacgaaaactcacgttaagggattttggtcatgcattctaggtactaaaacaattcatccagtaaaatataatattttattttctcccaatcaggcttgatccccagtaagtcaaaaaatagctcgacatactgttcttccccgatatcctccctgatcgaccggacgcagaaggcaatgtcataccacttgtccgccctgccgcttctcccaagatcaataaagccacttactttgccatctttcacaaagatgttgctgtctcccaggtcgccgtgggaaaagacaagttcctcttcgggcttttccgtctttaaaaaatcatacagctcgcgcggatctttaaatggagtgtcttcttcccagttttcgcaatccacatcggccagatcgttattcagtaagtaatccaattcggctaagcggctgtctaagctattcgtatagggacaatccgatatgtcgatggagtgaaagagcctgatgcactccgcatacagctcgataatcttttcagggctttgttcatcttcatactcttccgagcaaaggacgccatcggcctcactcatgagcagattgctccagccatcatgccgttcaaagtgcaggacctttggaacaggcagctttccttccagccatagcatcatgtccttttcccgttccacatcataggtggtccctttataccggctgtccgtcatttttaaatataggttttcattttctcccaccagcttatataccttagcaggagacattccttccgtatcttttacgcagcggtatttttcgatcagttttttcaattccggtgatattctcattttagccatttattatttccttcctcttttctacagtatttaaagataccccaagaagctaattataacaagacgaactccaattcactgttccttgcattctaaaaccttaaataccagaaaacagctttttcaaagttgttttcaaagttggcgtataacatagtatcgacggagccgattttgaaaccgcggtgatcacaggcagcaacgctctgtcatcgttacaatcaacatgctaccctccgcgagatcatccgtgtttcaaacccggcagcttagttgccgttcttccgaatagcatcggtaacatgagcaaagtctgccgccttacaacggctctcccgctgacgccgtcccggactgatgggctgcctgtatcgagtggtgattttgtgccgagctgccggtcggggagctgttggctggctggtggcaggatatattgtggtgtaaacaaattgacgcttagacaacttaataacacattgcggacgtttttaatgtactgaattaacgccgaattaattcgggggatctggattttagtactggattttggttttaggaattagaaattttattgatagaagtattttacaaatacaaatacatactaagggtttcttatatgctcaacacatgagcgaaaccctataggaaccctaattcccttatctgggaactactcacacattattatggagaaactcgagcttgtcgatcgacagatccggtcggcatctactctatttctttgccctcggacgagtgctggggcgtcggtttccactatcggcgagtacttctacacagccatcggtccagacggccgcgcttctgcgggcgatttgtgtacgcccgacagtcccggctccggatcggacgattgcgtcgcatcgaccctgcgcccaagctgcatcatcgaaattgccgtcaaccaagctctgatagagttggtcaagaccaatgcggagcatatacgcccggagtcgtggcgatcctgcaagctccggatgcctccgctcgaagtagcgcgtctgctgctccatacaagccaaccacggcctccagaagaagatgttggcgacctcgtattgggaatccccgaacatcgcctcgctccagtcaatgaccgctgttatgcggccattgtccgtcaggacattgttggagccgaaatccgcgtgcacgaggtgccggacttcggggcagtcctcggcccaaagcatcagctcatcgagagcctgcgcgacggacgcactgacggtgtcgtccatcacagtttgccagtgatacacatggggatcagcaatcgcgcatatgaaatcacgccatgtagtgtattgaccgattccttgcggtccgaatgggccgaacccgctcgtctggctaagatcggccgcagcgatcgcatccatagcctccgcgaccggttgtagaacagcgggcagttcggtttcaggcaggtcttgcaacgtgacaccctgtgcacggcgggagatgcaataggtcaggctctcgctaaactccccaatgtcaagcacttccggaatcgggagcgcggccgatgcaaagtgccgataaacataacgatctttgtagaaaccatcggcgcagctatttacccgcaggacatatccacgccctcctacatcgaagctgaaagcacgagattcttcgccctccgagagctgcatcaggtcggagacgctgtcgaacttttcgatcagaaacttctcgacagacgtcgcggtgagttcaggctttttcatatctcattgccccccgggatctgcgaaagctcgagagagatagatttgtagagagagactggtgatttcagcgtgtcctctccaaatgaaatgaacttccttatatagaggaaggtcttgcgaaggatagtgggattgtgcgtcatcccttacgtcagtggagatatcacatcaatccacttgctttgaagacgtggttggaacgtcttctttttccacgatgctcctcgtgggtgggggtccatctttgggaccactgtcggcagaggcatcttgaacgatagcctttcctttatcgcaatgatggcatttgtaggtgccaccttccttttctactgtccttttgatgaagtgacagatagctgggcaatggaatccgaggaggtttcccgatattaccctttgttgaaaagtctcaatagccctttggtcttctgagactgtatctttgatattcttggagtagacgagagtgtcgtgctccaccatgttatcacatcaatccacttgctttgaagacgtggttggaacgtcttctttttccacgatgctcctcgtgggtgggggtccatctttgggaccactgtcggcagaggcatcttgaacgatagcctttcctttatcgcaatgatggcatttgtaggtgccaccttccttttctactgtccttttgatgaagtgacagatagctgggcaatggaatccgaggaggtttcccgatattaccctttgttgaaaagtctcaatagccctttggtcttctgagactgtatctttgatattcttggagtagacgagagtgtcgtgctccaccatgttggcaagctgctctagccaatacgcaaaccgcctctccccgcgcgttggccgattcattaatgcagctggcacgacaggtttcccgactggaaagcgggcagtgagcgcaacgcaattaatgtgagttagctcactcattaggcaccccaggctttacactttatgcttccggctcgtatgttgtgtggaattgtgagcggataacaatttcacacaggaaacagctatgaccatgattacgaattctggcacgacaggtttcccgactggaaagcgggcagtgagcgcaacgcaattaatgtgagttagctcactcattaggcaccccaggctttacactttatgcttccggctcgtatgttgtgtggaattgtgagcggataacaatttcacacaggaaacagctatgaccatgattacgccaagcttgcatgcctgcaggtcaacatggtggagcacgacactctcgtctactccaagaatatcaaagatacagtctcagaagaccagagggctattgagacttttcaacaaagggtaatatcgggaaacctcctcggattccattgcccagctatctgtcacttcatcgaaaggacagtagaaaaggaagatggcttctacaaatgccatcattgcgataaaggaaaggctatcgttcaagatgcctctaccgacagtggtcccaaagatggacccccacccacgaggaacatcgtggaaaaagaagacgttccaaccacgtcttcaaagcaagtggattgatgtgatggtcaacatggtggagcacgacactctcgtctactccaagaatatcaaagatacagtctcagaagaccagagggctattgagacttttcaacaaagggtaatatcgggaaacctcctcggattccattgcccagctatctgtcacttcatcgaaaggacagtagaaaaggaagatggcttctacaaatgccatcattgcgataaaggaaaggctatcgttcaagatgcctctaccgacagtggtcccaaagatggacccccacccacgaggaacatcgtggaaaaagaagacgttccaaccacgtcttcaaagcaagtggattgatgtgatatctccactgacgtaagggatgacgcacaatcccactatccttcgcaagacccttcctctatataaggaagttcatttcatttggagaggcctgggtacctctaga

SEQ ID NO: 6 - DNA, 11926 bp, synthetic construct; identical to SEQ ID NO: 1
  source 1..11926: mol_type = other DNA

SEQ ID NO: 7 - DNA, 12652 bp, synthetic construct
  source 1..12652: mol_type = other DNA
gtaatcttaccactgtgtgtgtgtgtgtgtgtgtgtcgcgtcgtgtcgtgtcgtgttgtccgcacatttgagtcgtgctgtccgcaccttttctttcagtgtgttagaatacccgaggcatggctttccaaggtaccagcaggactttaactcaacagtcctcagcggctacgtctgacgaacttcaaaagatattatttagccctgaagccattaagaaaatggctgctgagtgtgacctaggccggcatcattggatgcgagctgataatgctatttcagtccggcccctcgttcccgaagtaacccacggtcgcattgtttctttctttaagtctgggtatgatgctggtgaattgtgctctaaaggatacatgagcgtccctcaagtgttgtgtgctgttactcgaacagtttccactgatgctgaagggtctctgagaatttacctagctgacttaggcgacaaggaattatctcccatagataagcaatgtgtcacattacataaccatgatctccccgctttagtgtctttccaaccgacgtatgattgtcctatggagacagttgggaatcggaagcggtgttttgctgtcgttattgagagacatggttacgttgggtataccggcaccacagctagcgtgtgtagtaattggcaagcacggttttcttctaagaataacaactacactcatatcgcagctgggaagactctagtactgccattcaatagattagctgagcaaacgaaaccgtcagccgtcgctcgcctattgaagtcgcaattgaataacatagaagcttcgcaatacgttttgacggattcgaagatcaatcagaatgcgcgcagtgagtccgaggaattaaatgttgagagccctcccgccgcaatcgggagttcttccgcgtcccgcttcgaaaccttcagaccgcaggtggttaacggtctttagattttcgtcgcgtattagtatataagtatgtgtgagtctgtacataatactatatctatagtgtcctgtgtgagttgatacagtagacaactgtgacgcgatgtcgtgttgagaagggaacacatctggttctagtaagccacatcattagttttgaggttcaattcctcttactccctgttgtgccccttactttttcatggatgcttctccacgaaattgcgtttcgtctactagatcaaggagtgtttgtgttgtgattttctctttgtgttgtagatatttgagtcgagtcatggacaaatctgaaactagtatggtgagcaagggcgaggagctgttcaccggggtggtgcccatcctggtcgagctggacggcgacgtaaacggccacaagttcagcgtgtccggcgagggcgagggcgatgccacctacggcaagctgaccctgaagttcatctgcaccaccggcaagctgcccgtgccctggcccaccctcgttaccaccttcacctacggcgtgcagtgcttcagccgctaccccgaccacatgaagcagcacgacttcttcaagtccgccatgcccgaaggctacgtccaggagcgcaccatcttcttcaaggacgacggcaactacaagacccgcgccgaggtgaagttcgagggcgacaccctggtgaaccgcatcgagctgaagggcatcgacttcaaggaggacggcaacatcctggggcacaagctggagtacaactacaacagccacaacgtctatatcatggccgacaagcagaagaacggcatcaaggtgaacttcaagatccgccacaacatcgaggacggcagcgtgcagctcgccgaccactaccagcagaacacccccatcggcgacggccccgtgctgctgcccgacaaccactacctgagcacccagtccgccctgagcaaagaccccaacgagaagcgcgatcacatggtcctgctggagttcgtgaccgccgccgggatcactcacggcatggacgagctgtacaaggggatcctcacgcgtgactacaaggacgacgatgacaaggcagattataaagatgatgacgataaacatcatcaccatcaccactgaacctgtgttttccagaaccctccctccgattctgtggcgggagctgagttggtagtgttgctataaactacctgaagtcactaaacgctatgcggtgaacgggttgtccatccagcttacggctaaaatggtcagtcgtggagaaatccacgccagtagacttacaagtctctgaggtgcctttgaaaccatctcctaggtttcttcggaaggacttcggtccgtgtacttctagcacaagatgctagtttagagtacgggcatcccccattttttttaatggggtctctcaaaggagaccaggatccgataccctgtcaccggatgtgttttccggtctgatgagtccgtgaggacgaaacaggactgtcctgcaggagctcgaattcggtacgctgaaatcaccagtctctctctacaaatctatctctctctattttctccataaataatgtgtgagtagtttccgataaggaaattagggttcttatagggtttcgtcatgtgttgagcatataagaaacccttagtatgtatttgtatttgtaaaatacttctatcaataaaatttctaattcctaaaaccaaaatcagtactaaatcagatccccaattcactggccgtcgttttacaacgtcgtgactgggaaaaccctggcgttacccaacttaatcgccttgcagcacatccccctttcgccagtggcactggccgtcgttttacaacgtcgtgactgggaaaaccctggcgttacccaacttaatcgccttgcagcacatccccctttcgccagctggcgtaatagcgaagaggcccgcaccgatcgcccttcccaacagttgcgcagcctgaatggcgaatgctagagcagcttgagcttggatcagattgtcgtttcccgccttcagtttaaactatcagtgtttgacaggatatattggcgggtaaacctaagagaaaagagcgtttattagaataacggatatttaaaagggcgtgaaaaggtttatccgttcgtccatttgtatgtgcatgccaaccacagggttcccctcgggatcaaagtactttgatccaacccctccgctgctatagtgcagtcggcttctgacgttcagtgcagccgtcttctgaaaacgacatgtcgcacaagtcctaagttacgcgacaggctgccgccctgcccttttcctggcgttttcttgtcgcgtgttttagtcgcataaagtagaatacttgcgactagaaccggagacattacgccatgaacaagagcgccgccgctggcctgctgggctatgcccgcgtcagcaccgacgaccaggacttgaccaaccaacgggccgaactgcacgcggccggctgcaccaagctgttttccgagaagatcaccggcaccaggcgcgaccgcccggagctggccaggatgcttgaccacctacgccctggcgacgttgtgacagtgaccaggctagaccgcctggcccgcagcacccgcgacctactggacattgccgagcgcatccaggaggccggcgcgggcctgcgtagcctggcagagccgtgggccgacaccaccacgccggccggccgcatggtgttgaccgtgttcgccggcattgccgagttcgagcgttccctaatcatcgaccgcacccggagcgggcgcgaggccgccaaggcccgaggcgtgaagtttggcccccgccctaccctcaccccggcacagatcgcgcacgcccgcgagctgatcgaccaggaaggccgcaccgtgaaagaggcggctgcactgcttggcgtgcatcgctcgaccctgtaccgcgcacttgagcgcagcgaggaagtgacgcccaccgaggccaggcggcgcggtgccttccgtgaggacgcattgaccgaggccgacgccctggcggccgccgagaatgaacgccaagaggaacaagcatgaaaccgcaccaggacggccaggacgaaccgtttttcattaccgaagagatcgaggcggagatgatcgcggccgggtacgtgttcgagccgcccgcgcacgtctcaaccgtgcggctgcatgaaatcctggccggtttgtctgatgccaagctggcggcctggccggccagcttggccgctgaagaaaccgagcgccgccgtctaaaaaggtgatgtgtatttgagtaaaacagcttgcgtcatgcggtcgctgcgtatatgatgcgatgagtaaataaacaaatacgcaaggggaacgcatgaaggttatcgctgtacttaaccagaaaggcgggtcaggcaagacgaccatcgcaacccatctagcccgcgccctgcaactcgccggggccgatgttctgttagtcgattccgatccccagggcagtgcccgcgattgggcggccgtgcgggaagatcaaccgctaaccgttgtcggcatcgaccgcccgacgattgaccgcgacgtgaaggccatcggccggcgcgacttcgtagtgatcgacggagcgccccaggcggcggacttggctgtgtccgcgatcaaggcagccgacttcgtgctgattccggtgcagccaagcccttacgacatatgggccaccgccgacctggtggagctggttaagcagcgcattgaggtcacggatggaaggctacaagcggcctttgtcgtgtcgcgggcgatcaaaggcacgcgcatcggcggtgaggttgccgaggcgctggccgggtacgagctgcccattcttgagtcccgtatcacgcagcgcgtgagctacccaggcactgccgccgccggcacaaccgttcttgaatcagaacccgagggcgacgctgcccgcgaggtccaggcgctggccgctgaaattaaatcaaaactcatttgagttaatgaggtaaagagaaaatgagcaaaagcacaaacacgctaagtgccggccgtccgagcgcacgcagcagcaaggctgcaacgttggccagcctggcagacacgccagccatgaagcgggtcaactttcagttgccggcggaggatcacaccaagctgaagatgtacgcggtacgccaaggcaagaccattaccgagctgctatctgaatacatcgcgcagctaccagagtaaatgagcaaatgaataaatgagtagatgaattttagcggctaaaggaggcggcatggaaaatcaagaacaaccaggcaccgacgccgtggaatgccccatgtgtggaggaacgggcggttggccaggcgtaagcggctgggttgtctgccggccctgcaatggcactggaacccccaagcccgaggaatcggcgtgacggtcgcaaaccatccggcccggtacaaatcggcgcggcgctgggtgatgacctggtggagaagttgaaggccgcgcaggccgcccagcggcaacgcatcgaggcagaagcacgccccggtgaatcgtggcaagcggccgctgatcgaatccgcaaagaatcccggcaaccgccggcagccggtgcgccgtcgattaggaagccgcccaagggcgacgagcaaccagattttttcgttccgatgctctatgacgtgggcacccgcgatagtcgcagcatcatggacgtggccgttttccgtctgtcgaagcgtgaccgacgagctggcgaggtgatccgctacgagcttccagacgggcacgtagaggtttccgcagggccggccggcatggccagtgtgtgggattacgacctggtactgatggcggtttcccatctaaccgaatccatgaaccgataccgggaagggaagggagacaagcccggccgcgtgttccgtccacacgttgcggacgtactcaagttctgccggcgagccgatggcggaaagcagaaagacgacctggtagaaacctgcattcggttaaacaccacgcacgttgccatgcagcgtacgaagaaggccaagaacggccgcctggtgacggtatccgagggtgaagccttgattagccgctacaagatcgtaaagagcgaaaccgggcggccggagtacatcgagatcgagctagctgattggatgtaccgcgagatcacagaaggcaagaacccggacgtgctgacggttcaccccgattactttttgatcgatcccggcatcggccgttttctctaccgcctggcacgccgcgccgcaggcaaggcagaagccagatggttgttcaagacgatctacgaacgcagtggcagcgccggagagttcaagaagttctgtttcaccgtgcgcaagctgatcgggtcaaatgacctgccggagtacgatttgaaggaggaggcggggcaggctggcccgatcctagtcatgcgctaccgcaacctgatcgagggcgaagcatccgccggttcctaatgtacggagcagatgctagggcaaattgccctagcaggggaaaaaggtcgaaaaggtctctttcctgtggatagcacgtacattgggaacccaaagccgtacattgggaaccggaacccgtacattgggaacccaaagccgtacattgggaaccggtcacacatgtaagtgactgatataaaagagaaaaaaggcgatttttccgcctaaaactctttaaaacttattaaaactcttaaaacccgcctggcctgtgcataactgtctggccagcgcacagccgaagagctgcaaaaagcgcctacccttcggtcgctgcgctccctacgccccgccgcttcgcgtcggcctatcgcggccgctggccgctcaaaaatggctggcctacggccaggcaatctaccagggcgcggacaagccgcgccgtcgccactcgaccgccggcgcccacatcaaggcaccctgcctcgcgcgtttcggtgatgacggtgaaaacctctgacacatgcagctcccggagacggtcacagcttgtctgtaagcggatgccgggagcagacaagcccgtcagggcgcgtcagcgggtgttggcgggtgtcggggcgcagccatgacccagtcacgtagcgatagcggagtgtatactggcttaactatgcggcatcagagcagattgtactgagagtgcaccatatgcggtgtgaaataccgcacagatgcgtaaggagaaaataccgcatcaggcgctcttccgcttcctcgctcactgactcgctgcgctcggtcgttcggctgcggcgagcggtatcagctcactcaaaggcggtaatacggttatccacagaatcaggggataacgcaggaaagaacatgtgagcaaaaggccagcaaaaggccaggaaccgtaaaaaggccgcgttgctggcgtttttccataggctccgcccccctgacgagcatcacaaaaatcgacgctcaagtcagaggtggcgaaacccgacaggactataaagataccaggcgtttccccctggaagctccctcgtgcgctctcctgttccgaccctgccgcttaccggatacctgtccgcctttctcccttcgggaagcgtggcgctttctcatagctcacgctgtaggtatctcagttcggtgtaggtcgttcgctccaagctgggctgtgtgcacgaaccccccgttcagcccgaccgctgcgccttatccggtaactatcgtcttgagtccaacccggtaagacacgacttatcgccactggcagcagccactggtaacaggattagcagagcgaggtatgtaggcggtgctacagagttcttgaagtggtggcctaactacggctacactagaaggacagtatttggtatctgcgctctgctgaagccagttaccttcggaaaaagagttggtagctcttgatccggcaaacaaaccaccgctggtagcggtggtttttttgtttgcaagcagcagattacgcgcagaaaaaaaggatctcaagaagatcctttgatcttttctacggggtctgacgctcagtggaacgaaaactcacgttaagggattttggtcatgcattctaggtactaaaacaattcatccagtaaaatataatattttattttctcccaatcaggcttgatccccagtaagtcaaaaaatagctcgacatactgttcttccccgatatcctccctgatcgaccggacgcagaaggcaatgtcataccacttgtccgccctgccgcttctcccaagatcaataaagccacttactttgccatctttcacaaagatgttgctgtctcccaggtcgccgtgggaaaagacaagttcctcttcgggcttttccgtctttaaaaaatcatacagctcgcgcggatctttaaatggagtgtcttcttcccagttttcgcaatccacatcggccagatcgttattcagtaagtaatccaattcggctaagcggctgtctaagctattcgtatagggacaatccgatatgtcgatggagtgaaagagcctgatgcactccgcatacagctcgataatcttttcagggctttgttcatcttcatactcttccgagcaaaggacgccatcggcctcactcatgagcagattgctccagccatcatgccgttcaaagtgcaggacctttggaacaggcagctttccttccagccatagcatcatgtccttttcccgttccacatcataggtggtccctttataccggctgtccgtcatttttaaatataggttttcattttctcccaccagcttatataccttagcaggagacattccttccgtatcttttacgcagcggtatttttcgatcagttttttcaattccggtgatattctcattttagccatttattatttccttcctcttttctacagtatttaaagataccccaagaagctaattataacaagacgaactccaattcactgttccttgcattctaaaaccttaaataccagaaaacagctttttcaaagttgttttcaaagttggcgtataacatagtatcgacggagccgattttgaaaccgcggtgatcacaggcagcaacgctctgtcatcgttacaatcaacatgctaccctccgcgagatcatccgtgtttcaaacccggcagcttagttgccgttcttccgaatagcatcggtaacatgagcaaagtctgccgccttacaacggctctcccgctgacgccgtcccggactgatgggctgcctgtatcgagtggtgattttgtgccgagctgccggtcggggagctgttggctggctggtggcaggatatattgtggtgtaaacaaattgacgcttagacaacttaataacacattgcggacgtttttaatgtactgaattaacgccgaattaattcgggggatctggattttagtactggattttggttttaggaattagaaattttattgatagaagtattttacaaatacaaatacatactaagggtttcttatatgctcaacacatgagcgaaaccctataggaaccctaattcccttatctgggaactactcacacattattatggagaaactcgagcttgtcgatcgacagatccggtcggcatctactctatttctttgccctcggacgagtgctggggcgtcggtttccactatcggcgagtacttctacacagccatcggtccagacggccgcgcttctgcgggcgatttgtgtacgcccgacagtcccggctccggatcggacgattgcgtcgcatcgaccctgcgcccaagctgcatcatcgaaattgccgtcaaccaagctctgatagagttggtcaagaccaatgcggagcatatacgcccggagtcgtggcgatcctgcaagctccggatgcctccgctcgaagtagcgcgtctgctgctccatacaagccaaccacggcctccagaagaagatgttggcgacctcgtattgggaatccccgaacatcgcctcgctccagtcaatgaccgctgttatgcggccattgtccgtcaggacattgttggagccgaaatccgcgtgcacgaggtgccggacttcggggcagtcctcggcccaaagcatcagctcatcgagagcctgcgcgacggacgcactgacggtgtcgtccatcacagtttgccagtgatacacatggggatcagcaatcgcgcatatgaaatcacgccatgtagtgtattgaccgattccttgcggtccgaatgggccgaacccgctcgtctggctaagatcggccgcagcgatcgcatccatagcctccgcgaccggttgtagaacagcgggcagttcggtttcaggcaggtcttgcaacgtgacaccctgtgcacggcgggagatgcaataggtcaggctctcgctaaactccccaatgtcaagcacttccggaatcgggagcgcggccgatgcaaagtgccgataaacataacgatctttgtagaaaccatcggcgcagctatttacccgcaggacatatccacgccctcctacatcgaagctgaaagcacgagattcttcgccctccgagagctgcatcaggtcggagacgctgtcgaacttttcgatcagaaacttctcgacagacgtcgcggtgagttcaggctttttcatatctcattgccccccgggatctgcgaaagctcgagagagatagatttgtagagagagactggtgatttcagcgtgtcctctccaaatgaaatgaacttccttatatagaggaaggtcttgcgaaggatagtgggattgtgcgtcatcccttacgtcagtggagatatcacatcaatccacttgctttgaagacgtggttggaacgtcttctttttccacgatgctcctcgtgggtgggggtccatctttgggaccactgtcggcagaggcatcttgaacgatagcctttcctttatcgcaatgatggcatttgtaggtgccaccttccttttctactgtccttttgatgaagtgacagatagctgggcaatggaatccgaggaggtttcccgatattaccctttgttgaaaagtctcaatagccctttggtcttctgagactgtatctttgatattcttggagtagacgagagtgtcgtgctccaccatgttatcacatcaatccacttgctttgaagacgtggttggaacgtcttctttttccacgatgctcctcgtgggtgggggtccatctttgggaccactgtcggcagaggcatcttgaacgatagcctttcctttatcgcaatgatggcatttgtaggtgccaccttccttttctactgtccttttgatgaagtgacagatagctgggcaatggaatccgaggaggtttcccgatattaccctttgttgaaaagtctcaatagccctttggtcttctgagactgtatctttgatattcttggagtagacgagagtgtcgtgctccaccatgttggcaagctgctctagccaatacgcaaaccgcctctccccgcgcgttggccgattcattaatgcagctggcacgacaggtttcccgactggaaagcgggcagtgagcgcaacgcaattaatgtgagttagctcactcattaggcaccccaggctttacactttatgcttccggctcgtatgttgtgtggaattgtgagcggataacaatttcacacaggaaacagctatgaccatgattacgaattctggcacgacaggtttcccgactggaaagcgggcagtgagcgcaacgcaattaatgtgagttagctcactcattaggcaccccaggctttacactttatgcttccggctcgtatgttgtgtggaattgtgagcggataacaatttcacacaggaaacagctatgaccatgattacgccaagcttgcatgcctgcaggtcaacatggtggagcacgacactctcgtctactccaagaatatcaaagatacagtctcagaagaccagagggctattgagacttttcaacaaagggtaatatcgggaaacctcctcggattccattgcccagctatctgtcacttcatcgaaaggacagtagaaaaggaagatggcttctacaaatgccatcattgcgataaaggaaaggctatcgttcaagatgcctctaccgacagtggtcccaaagatggacccccacccacgaggaacatcgtggaaaaagaagacgttccaaccacgtcttcaaagcaagtggattgatgtgatggtcaacatggtggagcacgacactctcgtctactccaagaatatcaaagatacagtctcagaagaccagagggctattgagacttttcaacaaagggtaatatcgggaaacctcctcggattccattgcccagctatctgtcacttcatcgaaaggacagtagaaaaggaagatggcttctacaaatgccatcattgcgataaaggaaaggctatcgttcaagatgcctctaccgacagtggtcccaaagatggacccccacccacgaggaacatcgtggaaaaagaagacgttccaaccacgtcttcaaagcaagtggattgatgtgatatctccactgacgtaagggatgacgcacaatcccactatccttcgcaagacccttcctctatataaggaagttcatttcatttggagaggcctgggtacctctaga

SEQ ID NO: 8 - DNA, 13622 bp, synthetic construct
  source 1..13622: mol_type = other DNA
gtttatttacaagagcgtacggttcaatccctgcctcccctgtaaaactaccctttgaaaacctctctttcttaatcttttctttgtaattcctatggcgacgtcctcgttcaacatcaatgaattggtagcctcccacggcgataaaggactactcgcgaccgccctcgttgataagacagctcatgagcagctcgaggagcaattacagcatcaacgtagaggccgtaaggtctacatccggaacgttttgggtgtaaaggattccgaggtcatccggaatcggtatggaggaaagtacgacctccatcttacccagcaggagtttgctccccacggcctagctggtgccctccgcttgtgtgaaactctcgattgtctagactctttcccttcatcaggtctgcggcaggacctcgtcttagacttcggaggaagttgggtcacacattacctccgcggacataacgtacactgttgttccccttgtttgggtatccgcgataagatgcgccatgcggaacgcttaatgaacatgcgcaagatcatcttgaacgatccacaacagttcgatggtcggcagccggatttctgcactcaaccggctgcggattgcaaagtacaagcccactttgctatatctattcatggaggttatgatatgggctttagaggattatgtgaagcgatgaatgctcacggaaccactattttgaagggaacgatgatgttcgatggtgcgatgatgtttgacgaccaaggtgtaatacccgaacttaattgtcagtggaggaagatcaggagtgctttctccgaaactgaagacgtcacaccactggttggtaagcttaattccacagttttctcccgcgtgcggaagttcaagacgatggtagcttttgatttcatcaacgagtctactatgtcttatgttcatgattgggagaatataaaatcttttcttacggaccagacttattcgtaccgagggatgacttacggtatcgaacgctgcgttatccacgctggtattatgacgtacaagattatcggtgtacctgggatgtgcccacccgaactcattcgacattgtatttggttcccctctattaaagactatgttggtctaaagatccccgcgtcgcaggatttggttgagtggaaaacagtgcggattttaacgtcaacattacgtgagactgaagagattgctatgaggtgttataatgataagaaagcgtggatggaacagttcaaggttatcctaggtgttctatccgcgaaatcatctaccattgttattaatggtatgtccatgcaatctggcgagcgaatagacattaatgattatcactacatcggtttcgccattcttcttcacacaaaaatgaagtacgaacaacttggaaaaatgtatgatatgtggaatgcttcgagtatttcgaagtggtttgccgcgttgactcgtccgctgcgtgtgtttttctccagtgttgttcacgcactattcccgactttgagaccccgcgaggaaaaagaatttttgatcaagctctccaccttcgtgacttttaatgaagagtgctcatttgacggtggagaggaatgggacgtgatatcatccgctgcatacgttgctacgcaggctgttaccgatgggaagattttggctgcgcagaaagccgagaagcttgctgagaagcttgcacaacccgtgagtgaggtatcggacagtcctgagacgtcatctcaaacgcctgatgatactgctgatgtttgtggaagggagcgagaggtttcggaactcgactccctatcagctcagacacgttcccccatcactagagttgctgaaagggctactgctatgttagagtatgccgcttatgagaaacaattgcacgacactacagtgtctaatttaaaacgtatttggaacatggcgggcggtgatgacaaaagaaactccctcgagggtaatttgaagtttgttttcgatacgtactttaccgttgatcctatggtgaacattcatttctccacgggtcggtggatgcgtcctgtgcccgagggtattgtttattctgtcggttataatgaacgcggtttaggtccgaagtctgatggagagctttacattgtcaatagtgaatgcgtgatctgtaacagtgaatctttatccactgtcacgcgttctcttcaagctccaaccgggaccattagtcaagttgacggagttgctggttgtgggaaaaccacggcaattaaatccatttttgagccgtccactgacatgatcgttaccgcgaacaagaagtccgcccaagatgtacgtatggcacttttcaaatcgtcggattccaaagaagcttgcacctttgttcgaacagccgattctgtcctacttaatgaatgtccgactgttagtagggttttggttgacgaggtcgttctgctacactttggtcaattatgtgccgtcatgtctaagttgaaggccgtgcgagctatatgttttggggattcggagcagattgccttttcctcgcgtgatgcttcatttgacatgcgtttctctaagattattcctgatgaaactagtgatgctgacaccacattccgtagcccacaagatgttgtaccgcttgtgcgtttaatggctacgaaggcccttccgaaaggaacccattcaaaatacacgaaatgggtttctcaatctaaagtgaaaagatctgttacatctcgtgccatcgctagtgtgacattggttgacttggattcttccaggttctatataacgatgacccaagctgataaggcctcactgatttcaagggcgaaagagatgaatctaccaaagactttctggaatgaaaggattaaaaccgtgcatgagtctcagggtatctccgaagaccacgttactttggtaagattaaagagtacaaaatgtgacctgtttaaacagttttcttattgtctcgttgcactgacgagacacaaggtcacattccgctacgagtactgtggtgtattgaacggcgatttaatcgccgaatgtgttgctcgtgcttagcggtctccctcttcgggcgggatctgagttggcggtaatctgcaaaccgtctgaagtcactaaacacattgtgtggtgaacgggttgtccatccagctaacggctaaaatggtcagtcgtggagaaatccacgccagtagacttacaagtctctgaggcacctttgaaaccatctcctaggtttcttcggaaggacttcggtccgtgtacttctagcacaacgtgctagtttcagggtacgggtgccccccactttcgtgggggtctctaaaaggagaccaggatccgataccctgtcaccggatgtgttttccggtctgatgagtccgtgaggacgaaacaggactgtcctgcaggagctcgaattcggtacgctgaaatcaccagtctctctctacaaatctatctctctctattttctccataaataatgtgtgagtagtttccgataaggaaattagggttcttatagggtttcgtcatgtgttgagcatataagaaacccttagtatgtatttgtatttgtaaaatacttctatcaataaaatttctaattcctaaaaccaaaatcagtactaaatcagatccccaattcactggccgtcgttttacaacgtcgtgactgggaaaaccctggcgttacccaacttaatcgccttgcagcacatccccctttcgccagtggcactggccgtcgttttacaacgtcgtgactgggaaaaccctggcgttacccaacttaatcgccttgcagcacatccccctttcgccagctggcgtaatagcgaagaggcccgcaccgatcgcccttcccaacagttgcgcagcctgaatggcgaatgctagagcagcttgagcttggatcagattgtcgtttcccgccttcagtttaaactatcagtgtttgacaggatatattggcgggtaaacctaagagaaaagagcgtttattagaataacggatatttaaaagggcgtgaaaaggtttatccgttcgtccatttgtatgtgcatgccaaccacagggttcccctcgggatcaaagtactttgatccaacccctccgctgctatagtgcagtcggcttctgacgttcagtgcagccgtcttctgaaaacgacatgtcgcacaagtcctaagttacgcgacaggctgccgccctgcccttttcctggcgttttcttgtcgcgtgttttagtcgcataaagtagaatacttgcgactagaaccggagacattacgccatgaacaagagcgccgccgctggcctgctgggctatgcccgcgtcagcaccgacgaccaggacttgaccaaccaacgggccgaactgcacgcggccggctgcaccaagctgttttccgagaagatcaccggcaccaggcgcgaccgcccggagctggccaggatgcttgaccacctacgccctggcgacgttgtgacagtgaccaggctagaccgcctggcccgcagcacccgcgacctactggacattgccgagcgcatccaggaggccggcgcgggcctgcgtagcctggcagagccgtgggccgacaccaccacgccggccggccgcatggtgttgaccgtgttcgccggcattgccgagttcgagcgttccctaatcatcgaccgcacccggagcgggcgcgaggccgccaaggcccgaggcgtgaagtttggcccccgccctaccctcaccccggcacagatcgcgcacgcccgcgagctgatcgaccaggaaggccgcaccgtgaaagaggcggctgcactgcttggcgtgcatcgctcgaccctgtaccgcgcacttgagcgcagcgaggaagtgacgcccaccgaggccaggcggcgcggtgccttccgtgaggacgcattgaccgaggccgacgccctggcggccgccgagaatgaacgccaagaggaacaagcatgaaaccgcaccaggacggccaggacgaaccgtttttcattaccgaagagatcgaggcggagatgatcgcggccgggtacgtgttcgagccgcccgcgcacgtctcaaccgtgcggctgcatgaaatcctggccggtttgtctgatgccaagctggcggcctggccggccagcttggccgctgaagaaaccgagcgccgccgtctaaaaaggtgatgtgtatttgagtaaaacagcttgcgtcatgcggtcgctgcgtatatgatgcgatgagtaaataaacaaatacgcaaggggaacgcatgaaggttatcgctgtacttaaccagaaaggcgggtcaggcaagacgaccatcgcaacccatctagcccgcgccctgcaactcgccggggccgatgttctgttagtcgattccgatccccagggcagtgcccgcgattgggcggccgtgcgggaagatcaaccgctaaccgttgtcggcatcgaccgcccgacgattgaccgcgacgtgaaggccatcggccggcgcgacttcgtagtgatcgacggagcgccccaggcggcggacttggctgtgtccgcgatcaaggcagccgacttcgtgctgattccggtgcagccaagcccttacgacatatgggccaccgccgacctggtggagctggttaagcagcgcattgaggtcacggatggaaggctacaagcggcctttgtcgtgtcgcgggcgatcaaaggcacgcgcatcggcggtgaggttgccgaggcgctggccgggtacgagctgcccattcttgagtcccgtatcacgcagcgcgtgagctacccaggcactgccgccgccggcacaaccgttcttgaatcagaacccgagggcgacgctgcccgcgaggtccaggcgctggccgctgaaattaaatcaaaactcatttgagttaatgaggtaaagagaaaatgagcaaaagcacaaacacgctaagtgccggccgtccgagcgcacgcagcagcaaggctgcaacgttggccagcctggcagacacgccagccatgaagcgggtcaactttcagttgccggcggaggatcacaccaagctgaagatgtacgcggtacgccaaggcaagaccattaccgagctgctatctgaatacatcgcgcagctaccagagtaaatgagcaaatgaataaatgagtagatgaattttagcggctaaaggaggcggcatggaaaatcaagaacaaccaggcaccgacgccgtggaatgccccatgtgtggaggaacgggcggttggccaggcgtaagcggctgggttgtctgccggccctgcaatggcactggaacccccaagcccgaggaatcggcgtgacggtcgcaaaccatccggcccggtacaaatcggcgcggcgctgggtgatgacctggtggagaagttgaaggccgcgcaggccgcccagcggcaacgcatcgaggcagaagcacgccccggtgaatcgtggcaagcggccgctgatcgaatccgcaaagaatcccggcaaccgccggcagccggtgcgccgtcgattaggaagccgcccaagggcgacgagcaaccagattttttcgttccgatgctctatgacgtgggcacccgcgatagtcgcagcatcatggacgtggccgttttccgtctgtcgaagcgtgaccgacgagctggcgaggtgatccgctacgagcttccagacgggcacgtagaggtttccgcagggccggccggcatggccagtgtgtgggattacgacctggtactgatggcggtttcccatctaaccgaatccatgaaccgataccgggaagggaagggagacaagcccggccgcgtgttccgtccacacgttgcggacgtactcaagttctgccggcgagccgatggcggaaagcagaaagacgacctggtagaaacctgcattcggttaaacaccacgcacgttgccatgcagcgtacgaagaaggccaagaacggccgcctggtgacggtatccgagggtgaagccttgattagccgctacaagatcgtaaagagcgaaaccgggcggccggagtacatcgagatcgagctagctgattggatgtaccgcgagatcacagaaggcaagaacccggacgtgctgacggttcaccccgattactttttgatcgatcccggcatcggccgttttctctaccgcctggcacgccgcgccgcaggcaaggcagaagccagatggttgttcaagacgatctacgaacgcagtggcagcgccggagagttcaagaagttctgtttcaccgtgcgcaagctgatcgggtcaaatgacctgccggagtacgatttgaaggaggaggcggggcaggctggcccgatcctagtcatgcgctaccgcaacctgatcgagggcgaagcatccgccggttcctaatgtacggagcagatgctagggcaaattgccctagcaggggaaaaaggtcgaaaaggtctctttcctgtggatagcacgtacattgggaacccaaagccgtacattgggaaccggaacccgtacattgggaacccaaagccgtacattgggaaccggtcacacatgtaagtgactgatataaaagagaaaaaaggcgatttttccgcctaaaactctttaaaacttattaaaactcttaaaacccgcctggcctgtgcataactgtctggccagcgcacagccgaagagctgcaaaaagcgcctacccttcggtcgctgcgctccctacgccccgccgcttcgcgtcggcctatcgcggccgctggccgctcaaaaatggctggcctacggccaggcaatctaccagggcgcggacaagccgcgccgtcgccactcgaccgccggcgcccacatcaaggcaccctgcctcgcgcgtttcggtgatgacggtgaaaacctctgacacatgcagctcccggagacggtcacagcttgtctgtaagcggatgccgggagcagacaagcccgtcagggcgcgtcagcgggtgttggcgggtgtcggggcgcagccatgacccagtcacgtagcgatagcggagtgtatactggcttaactatgcggcatcagagcagattgtactgagagtgcaccatatgcggtgtgaaataccgcacagatgcgtaaggagaaaataccgcatcaggcgctcttccgcttcctcgctcactgactcgctgcgctcggtcgttcggctgcggcgagcggtatcagctcactcaaaggcggtaatacggttatccacagaatcaggggataacgcaggaaagaacatgtgagcaaaaggccagcaaaaggccaggaaccgtaaaaaggccgcgttgctggcgtttttccataggctccgcccccctgacgagcatcacaaaaatcgacgctcaagtcagaggtggcgaaacccgacaggactataaagataccaggcgtttccccctggaagctccctcgtgcgctctcctgttccgaccctgccgcttaccggatacctgtccgcctttctcccttcgggaagcgtggcgctttctcatagctcacgctgtaggtatctcagttcggtgtaggtcgttcgctccaagctgggctgtgtgcacgaaccccccgttcagcccgaccgctgcgccttatccggtaactatcgtcttgagtccaacccggtaagacacgacttatcgccactggcagcagccactggtaacaggattagcagagcgaggtatgtaggcggtgctacagagttcttgaagtggtggcctaactacggctacactagaaggacagtatttggtatctgcgctctgctgaagccagttaccttcggaaaaagagttggtagctcttgatccggcaaacaaaccaccgctggtagcggtggtttttttgtttgcaagcagcagattacgcgcagaaaaaaaggatctcaagaagatcctttgatcttttctacggggtctgacgctcagtggaacgaaaactcacgttaagggattttggtcatgcattctaggtactaaaacaattcatccagtaaaatataatattttattttctcccaatcaggcttgatccccagtaagtcaaaaaatagctcgacatactgttcttccccgatatcctccctgatcgaccggacgcagaaggcaatgtcataccacttgtccgccctgccgcttctcccaagatcaataaagccacttactttgccatctttcacaaagatgttgctgtctcccaggtcgccgtgggaaaagacaagttcctcttcgggcttttccgtctttaaaaaatcatacagctcgcgcggatctttaaatggagtgtcttcttcccagttttcgcaatccacatcggccagatcgttattcagtaagtaatccaattcggctaagcggctgtctaagctattcgtatagggacaatccgatatgtcgatggagtgaaagagcctgatgcactccgcatacagctcgataatcttttcagggctttgttcatcttcatactcttccgagcaaaggacgccatcggcctcactcatgagcagattgctccagccatcatgccgttcaaagtgcaggacctttggaacaggcagctttccttccagccatagcatcatgtccttttcccgttccacatcataggtggtccctttataccggctgtccgtcatttttaaatataggttttcattttctcccaccagcttatataccttagcaggagacattccttccgtatcttttacgcagcggtatttttcgatcagttttttcaattccggtgatattctcattttagccatttattatttccttcctcttttctacagtatttaaagataccccaagaagctaattataacaagacgaactccaattcactgttccttgcattctaaaaccttaaataccagaaaacagctttttcaaagttgttttcaaagttggcgtataacatagtatcgacggagccgattttgaaaccgcggtgatcacaggcagcaacgctctgtcatcgttacaatcaacatgctaccctccgcgagatcatccgtgtttcaaacccggcagcttagttgccgttcttccgaatagcatcggtaacatgagcaaagtctgccgccttacaacggctctcccgctgacgccgtcccggactgatgggctgcctgtatcgagtggtgattttgtgccgagctgccggtcggggagctgttggctggctggtggcaggatatattgtggtgtaaacaaattgacgcttagacaacttaataacacattgcggacgtttttaatgtactgaattaacgccgaattaattcgggggatctggattttagtactggattttggttttaggaattagaaattttattgatagaagtattttacaaatacaaatacatactaagggtttcttatatgctcaacacatgagcgaaaccctataggaaccctaattcccttatctgggaactactcacacattattatggagaaactcgagcttgtcgatcgacagatccggtcggcatctactctatttctttgccctcggacgagtgctggggcgtcggtttccactatcggcgagtacttctacacagccatcggtccagacggccgcgcttctgcgggcgatttgtgtacgcccgacagtcccggctccggatcggacgattgcgtcgcatcgaccctgcgcccaagctgcatcatcgaaattgccgtcaaccaagctctgatagagttggtcaagaccaatgcggagcatatacgcccggagtcgtggcgatcctgcaagctccggatgcctccgctcgaagtagcgcgtctgctgctccatacaagccaaccacggcctccagaagaagatgttggcgacctcgtattgggaatccccgaacatcgcctcgctccagtcaatgaccgctgttatgcggccattgtccgtcaggacattgttggagccgaaatccgcgtgcacgaggtgccggacttcggggcagtcctcggcccaaagcatcagctcatcgagagcctgcgcgacggacgcactgacggtgtcgtccatcacagtttgccagtgatacacatggggatcagcaatcgcgcatatgaaatcacgccatgtagtgtattgaccgattccttgcggtccgaatgggccgaacccgctcgtctggctaagatcggccgcagcgatcgcatccatagcctccgcgaccggttgtagaacagcgggcagttcggtttcaggcaggtcttgcaacgtgacaccctgtgcacggcgggagatgcaataggtcaggctctcgctaaactccccaatgtcaagcacttccggaatcgggagcgcggccgatgcaaagtgccgataaacataacgatctttgtagaaaccatcggcgcagctatttacccgcaggacatatccacgccctcctacatcgaagctgaaagcacgagattcttcgccctccgagagctgcatcaggtcggagacgctgtcgaacttttcgatcagaaacttctcgacagacgtcgcggtgagttcaggctttttcatatctcattgccccccgggatctgcgaaagctcgagagagatagatttgtagagagagactggtgatttcagcgtgtcctctccaaatgaaatgaacttccttatatagaggaaggtcttgcgaaggatagtgggattgtgcgtcatcccttacgtcagtggagatatcacatcaatccacttgctttgaagacgtggttggaacgtcttctttttccacgatgctcctcgtgggtgggggtccatctttgggaccactgtcggcagaggcatcttgaacgatagcctttcctttatcgcaatgatggcatttgtaggtgccaccttccttttctactgtccttttgatgaagtgacagatagctgggcaatggaatccgaggaggtttcccgatattaccctttgttgaaaagtctcaatagccctttggtcttctgagactgtatctttgatattcttggagtagacgagagtgtcgtgctccaccatgttatcacatcaatccacttgctttgaagacgtggttggaacgtcttctttttccacgatgctcctcgtgggtgggggtccatctttgggaccactgtcggcagaggcatcttgaacgatagcctttcctttatcgcaatgatggcatttgtaggtgccaccttccttttctactgtccttttgatgaagtgacagatagctgggcaatggaatccgaggaggtttcccgatattaccctttgttgaaaagtctcaatagccctttggtcttctgagactgtatctttgatattcttggagtagacgagagtgtcgtgctccaccatgttggcaagctgctctagccaatacgcaaaccgcctctccccgcgcgttggccgattcattaatgcagctggcacgacaggtttcccgactggaaagcgggcagtgagcgcaacgcaattaatgtgagttagctcactcattaggcaccccaggctttacactttatgcttccggctcgtatgttgtgtggaattgtgagcggataacaatttcacacaggaaacagctatgaccatgattacgaattctggcacgacaggtttcccgactggaaagcgggcagtgagcgcaacgcaattaatgtgagttagctcactcattaggcaccccaggctttacactttatgcttccggctcgtatgttgtgtggaattgtgagcggataacaatttcacacaggaaacagctatgaccatgattacgccaagcttgcatgcctgcaggtcaacatggtggagcacgacactctcgtctactccaagaatatcaaagatacagtctcagaagaccagagggctattgagacttttcaacaaagggtaatatcgggaaacctcctcggattccattgcccagctatctgtcacttcatcgaaaggacagtagaaaaggaagatggcttctacaaatgccatcattgcgataaaggaaaggctatcgttcaagatgcctctaccgacagtggtcccaaagatggacccccacccacgaggaacatcgtggaaaaagaagacgttccaaccacgtcttcaaagcaagtggattgatgtgatggtcaacatggtggagcacgacactctcgtctactccaagaatatcaaagatacagtctcagaagaccagagggctattgagacttttcaacaaagggtaatatcgggaaacctcctcggattccattgcccagctatctgtcacttcatcgaaaggacagtagaaaaggaagatggcttctacaaatgccatcattgcgataaaggaaaggctatcgttcaagatgcctctaccgacagtggtcccaaagatggacccccacccacgaggaacatcgtggaaaaagaagacgttccaaccacgtcttcaaagcaagtggattgatgtgatatctccactgacgtaagggatgacgcacaatcccactatccttcgcaagacccttcctctatataaggaagttcatttcatttggagaggcctgggtacc

SEQ ID NO: 9 - DNA, 13321 bp, synthetic construct
  source 1..13321: mol_type = other DNA
gtttatttacaagagcgtacggttcaacccctgcctcccctgtaaaactccctagacttaaatcttttctttctagtatcttttctatggctttccctgcccccgcattctcactagccaatcttttgaacggcagttacggtgtcgacactcccgaggatgtggaacgtttgcgatctgagcaacgcgaagaggctgctgcggcctgtcgtaattacaggcccctacccgctgtggatgtcagcgagagtgtcacagaggacgcgcattccctccgaactcctgacggagctcccgctgaagcggtgtctgatgagtttgtaacttatggtgctgaagattaccttgaaaaatctgatgatgagctccttgtcgcttttgagacgatggtcaaacccatgcgtatcggacaactatggtgccctgcgtttaataaatgttcttttatttccagcattgctatggccagagctttgttgttggcacctagaacatcccaccgaaccatgaagtgttttgaagacctggtcgcggctatttacactaaatctgatttctactacagtgaagagtgtgaagccgacgacgctcagatagatatctcgtctcgcgatgtacccggttattctttcgaaccgtggtcccgaacgtctggatttgaaccgccgcccatttgtgaagcgtgcgacatgatcatgtaccagtgcccgtgttttgattttaatgctttaaagaaatcgtgcgctgagaggaccttcgctgatgattatgttattgaaggtttagatggtgttgttgataatgcgactctgttgtcgaatttgggtccatttttggtacccgtgaagtgtcaatatgaaaaatgtccaacgccaaccatcgcgattcctccggatttaaaccgtgctactgatcgtgttgatatcaatttagttcaatccatttgtgactcgactctgcccactcatagtaattacgacgactcttttcatcaagtgttcgtcgaaagtgcagactattctatagatctggatcatgttagacttcgacagtctgatcttattgcaaaaattccagattcagggcatatgataccggttctgaacaccgggagcggtcacaagagagtaggtacaacgaaggaggtccttacagcaattaagaaacgtaatgctgacgttccagagctaggtgattccgttaatttgtctagattgagtaaagctgtggctgagagattcttcatttcatacatcaatggtaactctctagcatccagtaactttgtcaatgtcgttagtaacttccacgattacatggaaaaatggaagtcctcaggtctttcttatgatgatcttccggatcttcatgctgagaatttgcagttttatgaccacatgataaaatccgatgtgaaacctgtggtgagcgacacactcaatatcgacagaccggttccagctactataacgtatcataagaagagtataacctcccagttctcaccgttattcacagcgctattcgagcgcttccagagatgccttcgagaacgtattattcttcctgttggtaagatttcatcccttgagatggcaggatttgatgtcaagaacaagcactgcctcgagattgacctgtctaagtttgataagtctcaaggtgaatttcacttgctaatccaggaacacattttgaatggtctaggatgtccagctccgataactaagtggtggtgtgatttccatcgattctcttacattagagaccgtagagctggtgttggtatgcctattagtttccagagacgaactggcgatgcactcacttattttggcaataccatcgtcaccatggctgagtttgcctggtgttatgacaccgaccaattcgaaaagcttttattctcaggcgatgattctctaggattttcactgcttccccctgttggtgacccgagtaaattcacaactcttttcaacatggaagctaaggtgatggaacctgccgtaccatatatttgttcgaagttcttactctctgacgagttcggtaacacattttccgttccagatccattgcgcgaggttcagcggttaggaacaaagaaaattccctattctgacaatgatgaattcttgtttgctcacttcatgagctttgttgatcgattgaagtttttggaccgaatgtctcagtcgtgtatcgatcaactttcgattttcttcgaattgaaatacaagaagtctggggaagaggctgctttaatgttaggcgcctttaagaagtataccgctaatttccagtcctacaaagaactctattattcagatcgtcgtcagtgcgaattgatcaattcgttttgtagtacagagttcagggttgagcgtgtaaattccaacaaacagcgaaagaattatggaattgaacgtaggtgcaatgacaaacgtcgaactccaactggctcgtatggtggaggcgaagaagcagagacgaaggtctcacaaacagaatcgacgggaacgaggtcacaaaagtcccagcgagagagcgcgttcaaatctcagactattccgcttcctaccgttctatcaagtggatggttcggaactgacagggtcatgccgccatgtgaacgtggcggagttacccgagtctgaggcctctcgtttagagttatcggcggaagaccatgattttgacgatacagattggttcgccggtaacgaatgggcggaaggtgctttctgaaacctccccttccgcatctccctccggttttctgtggcgggagctgagttggcagtattgctataaactgtctgaagtcactaaacacattgtggtgaacgggttgtccatccagcttacggctaaaatggtcagtcgtagaggaatctacgccagcagacttacaagtctctgaggcacctttgaaaccatctcctaggtttcttcggaaggacttcggtccgtgtacttctagcacaacgtgctagtttcagggtacgggtgccccccacttttgtggggcctccaaaaggagaccaggatccgataccctgtcaccggatgtgttttccggtctgatgagtccgtgaggacgaaacaggactgtcctgcaggagctcgaattcggtacgctgaaatcaccagtctctctctacaaatctatctctctctattttctccataaataatgtgtgagtagtttccgataaggaaattagggttcttatagggtttcgtcatgtgttgagcatataagaaacccttagtatgtatttgtatttgtaaaatacttctatcaataaaatttctaattcctaaaaccaaaatcagtactaaatcagatccccaattcactggccgtcgttttacaacgtcgtgactgggaaaaccctggcgttacccaacttaatcgccttgcagcacatccccctttcgccagtggcactggccgtcgttttacaacgtcgtgactgggaaaaccctggcgttacccaacttaatcgccttgcagcacatccccctttcgccagctggcgtaatagcgaagaggcccgcaccgatcgcccttcccaacagttgcgcagcctgaatggcgaatgctagagcagcttgagcttggatcagattgtcgtttcccgccttcagtttaaactatcagtgtttgacaggatatattggcgggtaaacctaagagaaaagagcgtttattagaataacggatatttaaaagggcgtgaaaaggtttatccgttcgtccatttgtatgtgcatgccaaccacagggttcccctcgggatcaaagtactttgatccaacccctccgctgctatagtgcagtcggcttctgacgttcagtgcagccgtcttctgaaaacgacatgtcgcacaagtcctaagttacgcgacaggctgccgccctgcccttttcctggcgttttcttgtcgcgtgttttagtcgcataaagtagaatacttgcgactagaaccggagacattacgccatgaacaagagcgccgccgctggcctgctgggctatgcccgcgtcagcaccgacgaccaggacttgaccaaccaacgggccgaactgcacgcggccggctgcaccaagctgttttccgagaagatcaccggcaccaggcgcgaccgcccggagctggccaggatgcttgaccacctacgccctggcgacgttgtgacagtgaccaggctagaccgcctggcccgcagcacccgcgacctactggacattgccgagcgcatccaggaggccggcgcgggcctgcgtagcctggcagagccgtgggccgacaccaccacgccggccggccgcatggtgttgaccgtgttcgccggcattgccgagttcgagcgttccctaatcatcgaccgcacccggagcgggcgcgaggccgccaaggcccgaggcgtgaagtttggcccccgccctaccctcaccccggcacagatcgcgcacgcccgcgagctgatcgaccaggaaggccgcaccgtgaaagaggcggctgcactgcttggcgtgcatcgctcgaccctgtaccgcgcacttgagcgcagcgaggaagtgacgcccaccgaggccaggcggcgcggtgccttccgtgaggacgcattgaccgaggccgacgccctggcggccgccgagaatgaacgccaagaggaacaagcatgaaaccgcaccaggacggccaggacgaaccgtttttcattaccgaagagatcgaggcggagatgatcgcggccgggtacgtgttcgagccgcccgcgcacgtctcaaccgtgcggctgcatgaaatcctggccggtttgtctgatgccaagctggcggcctggccggccagcttggccgctgaagaaaccgagcgccgccgtctaaaaaggtgatgtgtatttgagtaaaacagcttgcgtcatgcggtcgctgcgtatatgatgcgatgagtaaataaacaaatacgcaaggggaacgcatgaaggttatcgctgtacttaaccagaaaggcgggtcaggcaagacgaccatcgcaacccatctagcccgcgccctgcaactcgccggggccgatgttctgttagtcgattccgatccccagggcagtgcccgcgattgggcggccgtgcgggaagatcaaccgctaaccgttgtcggcatcgaccgcccgacgattgaccgcgacgtgaaggccatcggccggcgcgacttcgtagtgatcgacggagcgccccaggcggcggacttggctgtgtccgcgatcaaggcagccgacttcgtgctgattccggtgcagccaagcccttacgacatatgggccaccgccgacctggtggagctggttaagcagcgcattgaggtcacggatggaaggctacaagcggcctttgtcgtgtcgcgggcgatcaaaggcacgcgcatcggcggtgaggttgccgaggcgctggccgggtacgagctgcccattcttgagtcccgtatcacgcagcgcgtgagctacccaggcactgccgccgccggcacaaccgttcttgaatcagaacccgagggcgacgctgcccgcgaggtccaggcgctggccgctgaaattaaatcaaaactcatttgagttaatgaggtaaagagaaaatgagcaaaagcacaaacacgctaagtgccggccgtccgagcgcacgcagcagcaaggctgcaacgttggccagcctggcagacacgccagccatgaagcgggtcaactttcagttgccggcggaggatcacaccaagctgaagatgtacgcggtacgccaaggcaagaccattaccgagctgctatctgaatacatcgcgcagctaccagagtaaatgagcaaatgaataaatgagtagatgaattttagcggctaaaggaggcggcatggaaaatcaagaacaaccaggcaccgacgccgtggaatgccccatgtgtggaggaacgggcggttggccaggcgtaagcggctgggttgtctgccggccctgcaatggcactggaacccccaagcccgaggaatcggcgtgacggtcgcaaaccatccggcccggtacaaatcggcgcggcgctgggtgatgacctggtggagaagttgaaggccgcgcaggccgcccagcggcaacgcatcgaggcagaagcacgccccggtgaatcgtggcaagcggccgctgatcgaatccgcaaagaatcccggcaaccgccggcagccggtgcgccgtcgattaggaagccgcccaagggcgacgagcaaccagattttttcgttccgatgctctatgacgtgggcacccgcgatagtcgcagcatcatggacgtggccgttttccgtctgtcgaagcgtgaccgacgagctggcgaggtgatccgctacgagcttccagacgggcacgtagaggtttccgcagggccggccggcatggccagtgtgtgggattacgacctggtactgatggcggtttcccatctaaccgaatccatgaaccgataccgggaagggaagggagacaagcccggccgcgtgttccgtccacacgttgcggacgtactcaagttctgccggcgagccgatggcggaaagcagaaagacgacctggtagaaacctgcattcggttaaacaccacgcacgttgccatgcagcgtacgaagaaggccaagaacggccgcctggtgacggtatccgagggtgaagccttgattagccgctacaagatcgtaaagagcgaaaccgggcggccggagtacatcgagatcgagctagctgattggatgtaccgcgagatcacagaaggcaagaacccggacgtgctgacggttcaccccgattactttttgatcgatcccggcatcggccgttttctctaccgcctggcacgccgcgccgcaggcaaggcagaagccagatggttgttcaagacgatctacgaacgcagtggcagcgccggagagttcaagaagttctgtttcaccgtgcgcaagctgatcgggtcaaatgacctgccggagtacgatttgaaggaggaggcggggcaggctggcccgatcctagtcatgcgctaccgcaacctgatcgagggcgaagcatccgccggttcctaatgtacggagcagatgctagggcaaattgccctagcaggggaaaaaggtcgaaaaggtctctttcctgtggatagcacgtacattgggaacccaaagccgtacattgggaaccggaacccgtacattgggaacccaaagccgtacattgggaaccggtcacacatgtaagtgactgatataaaagagaaaaaaggcgatttttccgcctaaaactctttaaaacttattaaaactcttaaaacccgcctggcctgtgcataactgtctggccagcgcacagccgaagagctgcaaaaagcgcctacccttcggtcgctgcgctccctacgccccgccgcttcgcgtcggcctatcgcggccgctggccgctcaaaaatggctggcctacggccaggcaatctaccagggcgcggacaagccgcgccgtcgccactcgaccgccggcgcccacatcaaggcaccctgcctcgcgcgtttcggtgatgacggtgaaaacctctgacacatgcagctcccggagacggtcacagcttgtctgtaagcggatgccgggagcagacaagcccgtcagggcgcgtcagcgggtgttggcgggtgtcggggcgcagccatgacccagtcacgtagcgatagcggagtgtatactggcttaactatgcggcatcagagcagattgtactgagagtgcaccatatgcggtgtgaaataccgcacagatgcgtaaggagaaaataccgcatcaggcgctcttccgcttcctcgctcactgactcgctgcgctcggtcgttcggctgcggcgagcggtatcagctcactcaaaggcggtaatacggttatccacagaatcaggggataacgcaggaaagaacatgtgagcaaaaggccagcaaaaggccaggaaccgtaaaaaggccgcgttgctggcgtttttccataggctccgcccccctgacgagcatcacaaaaatcgacgctcaagtcagaggtggcgaaacccgacaggactataaagataccaggcgtttccccctggaagctccctcgtgcgctctcctgttccgaccctgccgcttaccggatacctgtccgcctttctcccttcgggaagcgtggcgctttctcatagctcacgctgtaggtatctcagttcggtgtaggtcgttcgctccaagctgggctgtgtgcacgaaccccccgttcagcccgaccgctgcgccttatccggtaactatcgtcttgagtccaacccggtaagacacgacttatcgccactggcagcagccactggtaacaggattagcagagcgaggtatgtaggcggtgctacagagttcttgaagtggtggcctaactacggctacactagaaggacagtatttggtatctgcgctctgctgaagccagttaccttcggaaaaagagttggtagctcttgatccggcaaacaaaccaccgctggtagcggtggtttttttgtttgcaagcagcagattacgcgcagaaaaaaaggatctcaagaagatcctttgatcttttctacggggtctgacgctcagtggaacgaaaactcacgttaagggattttggtcatgcattctaggtactaaaacaattcatccagtaaaatataatattttattttctcccaatcaggcttgatccccagtaagtcaaaaaatagctcgacatactgttcttccccgatatcctccctgatcgaccggacgcagaaggcaatgtcataccacttgtccgccctgccgcttctcccaagatcaataaagccacttactttgccatctttcacaaagatgttgctgtctcccaggtcgccgtgggaaaagacaagttcctcttcgggcttttccgtctttaaaaaatcatacagctcgcgcggatctttaaatggagtgtcttcttcccagttttcgcaatccacatcggccagatcgttattcagtaagtaatccaattcggctaagcggctgtctaagctattcgtatagggacaatccgatatgtcgatggagtgaaagagcctgatgcactccgcatacagctcgataatcttttcagggctttgttcatcttcatactcttccgagcaaaggacgccatcggcctcactcatgagcagattgctccagccatcatgccgttcaaagtgcaggacctttggaacaggcagctttccttccagccatagcatcatgtccttttcccgttccacatcataggtggtccctttataccggctgtccgtcatttttaaatataggttttcattttctcccaccagcttatataccttagcaggagacattccttccgtatcttttacgcagcggtatttttcgatcagttttttcaattccggtgatattctcattttagccatttattatttccttcctcttttctacagtatttaaagataccccaagaagctaattataacaagacgaactccaattcactgttccttgcattctaaaaccttaaataccagaaaacagctttttcaaagttgttttcaaagttggcgtataacatagtatcgacggagccgattttgaaaccgcggtgatcacaggcagcaacgctctgtcatcgttacaatcaacatgctaccctccgcgagatcatccgtgtttcaaacccggcagcttagttgccgttcttccgaatagcatcggtaacatgagcaaagtctgccgccttacaacggctctcccgctgacgccgtcccggactgatgggctgcctgtatcgagtggtgattttgtgccgagctgccggtcggggagctgttggctggctggtggcaggatatattgtggtgtaaacaaattgacgcttagacaacttaataacacattgcggacgtttttaatgtactgaattaacgccgaattaattcgggggatctggattttagtactggattttggttttaggaattagaaattttattgatagaagtattttacaaatacaaatacatactaagggtttcttatatgctcaacacatgagcgaaaccctataggaaccctaattcccttatctgggaactactcacacattattatggagaaactcgagcttgtcgatcgacagatccggtcggcatctactctatttctttgccctcggacgagtgctggggcgtcggtttccactatcggcgagtacttctacacagccatcggtccagacggccgcgcttctgcgggcgatttgtgtacgcccgacagtcccggctccggatcggacgattgcgtcgcatcgaccctgcgcccaagctgcatcatcgaaattgccgtcaaccaagctctgatagagttggtcaagaccaatgcggagcatatacgcccggagtcgtggcgatcctgcaagctccggatgcctccgctcgaagtagcgcgtctgctgctccatacaagccaaccacggcctccagaagaagatgttggcgacctcgtattgggaatccccgaacatcgcctcgctccagtcaatgaccgctgttatgcggccattgtccgtcaggacattgttggagccgaaatccgcgtgcacgaggtgccggacttcggggcagtcctcggcccaaagcatcagctcatcgagagcctgcgcgacggacgcactgacggtgtcgtccatcacagtttgccagtgatacacatggggatcagcaatcgcgcatatgaaatcacgccatgtagtgtattgaccgattccttgcggtccgaatgggccgaacccgctcgtctggctaagatcggccgcagcgatcgcatccatagcctccgcgaccggttgtagaacagcgggcagttcggtttcaggcaggtcttgcaacgtgacaccctgtgcacggcgggagatgcaataggtcaggctctcgctaaactccccaatgtcaagcacttccggaatcgggagcgcggccgatgcaaagtgccgataaacataacgatctttgtagaaaccatcggcgcagctatttacccgcaggacatatccacgccctcctacatcgaagctgaaagcacgagattcttcgccctccgagagctgcatcaggtcggagacgctgtcgaacttttcgatcagaaacttctcgacagacgtcgcggtgagttcaggctttttcatatctcattgccccccgggatctgcgaaagctcgagagagatagatttgtagagagagactggtgatttcagcgtgtcctctccaaatgaaatgaacttccttatatagaggaaggtcttgcgaaggatagtgggattgtgcgtcatcccttacgtcagtggagatatcacatcaatccacttgctttgaagacgtggttggaacgtcttctttttccacgatgctcctcgtgggtgggggtccatctttgggaccactgtcggcagaggcatcttgaacgatagcctttcctttatcgcaatgatggcatttgtaggtgccaccttccttttctactgtccttttgatgaagtgacagatagctgggcaatggaatccgaggaggtttcccgatattaccctttgttgaaaagtctcaatagccctttggtcttctgagactgtatctttgatattcttggagtagacgagagtgtcgtgctccaccatgttatcacatcaatccacttgctttgaagacgtggttggaacgtcttctttttccacgatgctcctcgtgggtgggggtccatctttgggaccactgtcggcagaggcatcttgaacgatagcctttcctttatcgcaatgatggcatttgtaggtgccaccttccttttctactgtccttttgatgaagtgacagatagctgggcaatggaatccgaggaggtttcccgatattaccctttgttgaaaagtctcaatagccctttggtcttctgagactgtatctttgatattcttggagtagacgagagtgtcgtgctccaccatgttggcaagctgctctagccaatacgcaaaccgcctctccccgcgcgttggccgattcattaatgcagctggcacgacaggtttcccgactggaaagcgggcagtgagcgcaacgcaattaatgtgagttagctcactcattaggcaccccaggctttacactttatgcttccggctcgtatgttgtgtggaattgtgagcggataacaatttcacacaggaaacagctatgaccatgattacgaattctggcacgacaggtttcccgactggaaagcgggcagtgagcgcaacgcaattaatgtgagttagctcactcattaggcaccccaggctttacactttatgcttccggctcgtatgttgtgtggaattgtgagcggataacaatttcacacaggaaacagctatgaccatgattacgccaagcttgcatgcctgcaggtcaacatggtggagcacgacactctcgtctactccaagaatatcaaagatacagtctcagaagaccagagggctattgagacttttcaacaaagggtaatatcgggaaacctcctcggattccattgcccagctatctgtcacttcatcgaaaggacagtagaaaaggaagatggcttctacaaatgccatcattgcgataaaggaaaggctatcgttcaagatgcctctaccgacagtggtcccaaagatggacccccacccacgaggaacatcgtggaaaaagaagacgttccaaccacgtcttcaaagcaagtggattgatgtgatggtcaacatggtggagcacgacactctcgtctactccaagaatatcaaagatacagtctcagaagaccagagggctattgagacttttcaacaaagggtaatatcgggaaacctcctcggattccattgcccagctatctgtcacttcatcgaaaggacagtagaaaaggaagatggcttctacaaatgccatcattgcgataaaggaaaggctatcgttcaagatgcctctaccgacagtggtcccaaagatggacccccacccacgaggaacatcgtggaaaaagaagacgttccaaccacgtcttcaaagcaagtggattgatgtgatatctccactgacgtaagggatgacgcacaatcccactatccttcgcaagacccttcctctatataaggaagttcatttcatttggagaggcctgggtacctctaga

SEQ ID NO: 10 - DNA, 11178 bp, synthetic construct
  source 1..11178: mol_type = other DNA
agtactttgatccaacccctccgctgctatagtgcagtcggcttctgacgttcagtgcagccgtcttctgaaaacgacatgtcgcacaagtcctaagttacgcgacaggctgccgccctgcccttttcctggcgttttcttgtcgcgtgttttagtcgcataaagtagaatacttgcgactagaaccggagacattacgccatgaacaagagcgccgccgctggcctgctgggctatgcccgcgtcagcaccgacgaccaggacttgaccaaccaacgggccgaactgcacgcggccggctgcaccaagctgttttccgagaagatcaccggcaccaggcgcgaccgcccggagctggccaggatgcttgaccacctacgccctggcgacgttgtgacagtgaccaggctagaccgcctggcccgcagcacccgcgacctactggacattgccgagcgcatccaggaggccggcgcgggcctgcgtagcctggcagagccgtgggccgacaccaccacgccggccggccgcatggtgttgaccgtgttcgccggcattgccgagttcgagcgttccctaatcatcgaccgcacccggagcgggcgcgaggccgccaaggcccgaggcgtgaagtttggcccccgccctaccctcaccccggcacagatcgcgcacgcccgcgagctgatcgaccaggaaggccgcaccgtgaaagaggcggctgcactgcttggcgtgcatcgctcgaccctgtaccgcgcacttgagcgcagcgaggaagtgacgcccaccgaggccaggcggcgcggtgccttccgtgaggacgcattgaccgaggccgacgccctggcggccgccgagaatgaacgccaagaggaacaagcatgaaaccgcaccaggacggccaggacgaaccgtttttcattaccgaagagatcgaggcggagatgatcgcggccgggtacgtgttcgagccgcccgcgcacgtctcaaccgtgcggctgcatgaaatcctggccggtttgtctgatgccaagctggcggcctggccggccagcttggccgctgaagaaaccgagcgccgccgtctaaaaaggtgatgtgtatttgagtaaaacagcttgcgtcatgcggtcgctgcgtatatgatgcgatgagtaaataaacaaatacgcaaggggaacgcatgaaggttatcgctgtacttaaccagaaaggcgggtcaggcaagacgaccatcgcaacccatctagcccgcgccctgcaactcgccggggccgatgttctgttagtcgattccgatccccagggcagtgcccgcgattgggcggccgtgcgggaagatcaaccgctaaccgttgtcggcatcgaccgcccgacgattgaccgcgacgtgaaggccatcggccggcgcgacttcgtagtgatcgacggagcgccccaggcggcggacttggctgtgtccgcgatcaaggcagccgacttcgtgctgattccggtgcagccaagcccttacgacatatgggccaccgccgacctggtggagctggttaagcagcgcattgaggtcacggatggaaggctacaagcggcctttgtcgtgtcgcgggcgatcaaaggcacgcgcatcggcggtgaggttgccgaggcgctggccgggtacgagctgcccattcttgagtcccgtatcacgcagcgcgtgagctacccaggcactgccgccgccggcacaaccgttcttgaatcagaacccgagggcgacgctgcccgcgaggtccaggcgctggccgctgaaattaaatcaaaactcatttgagttaatgaggtaaagagaaaatgagcaaaagcacaaacacgctaagtgccggccgtccgagcgcacgcagcagcaaggctgcaacgttggccagcctggcagacacgccagccatgaagcgggtcaactttcagttgccggcggaggatcacaccaagctgaagatgtacgcggtacgccaaggcaagaccattaccgagctgctatctgaatacatcgcgcagctaccagagtaaatgagcaaatgaataaatgagtagatgaattttagcggctaaaggaggcggcatggaaaatcaagaacaaccaggcaccgacgccgtggaatgccccatgtgtggaggaacgggcggttggccaggcgtaagcggctgggttgtctgccggccctgcaatggcactggaacccccaagcccgaggaatcggcgtgacggtcgcaaaccatccggcccggtacaaatcggcgcggcgctgggtgatgacctggtggagaagttgaaggccgcgcaggccgcccagcggcaacgcatcgaggcagaagcacgccccggtgaatcgtggcaagcggccgctgatcgaatccgcaaagaatcccggcaaccgccggcagccggtgcgccgtcgattaggaagccgcccaagggcgacgagcaaccagattttttcgttccgatgctctatgacgtgggcacccgcgatagtcgcagcatcatggacgtggccgttttccgtctgtcgaagcgtgaccgacgagctggcgaggtgatccgctacgagcttccagacgggcacgtagaggtttccgcagggccggccggcatggccagtgtgtgggattacgacctggtactgatggcggtttcccatctaaccgaatccatgaaccgataccgggaagggaagggagacaagcccggccgcgtgttccgtccacacgttgcggacgtactcaagttctgccggcgagccgatggcggaaagcagaaagacgacctggtagaaacctgcattcggttaaacaccacgcacgttgccatgcagcgtacgaagaaggccaagaacggccgcctggtgacggtatccgagggtgaagccttgattagccgctacaagatcgtaaagagcgaaaccgggcggccggagtacatcgagatcgagctagctgattggatgtaccgcgagatcacagaaggcaagaacccggacgtgctgacggttcaccccgattactttttgatcgatcccggcatcggccgttttctctaccgcctggcacgccgcgccgcaggcaaggcagaagccagatggttgttcaagacgatctacgaacgcagtggcagcgccggagagttcaagaagttctgtttcaccgtgcgcaagctgatcgggtcaaatgacctgccggagtacgatttgaaggaggaggcggggcaggctggcccgatcctagtcatgcgctaccgcaacctgatcgagggcgaagcatccgccggttcctaatgtacggagcagatgctagggcaaattgccctagcaggggaaaaaggtcgaaaaggtctctttcctgtggatagcacgtacattgggaacccaaagccgtacattgggaaccggaacccgtacattgggaacccaaagccgtacattgggaaccggtcacacatgtaagtgactgatataaaagagaaaaaaggcgatttttccgcctaaaactctttaaaacttattaaaactcttaaaacccgcctggcctgtgcataactgtctggccagcgcacagccgaagagctgcaaaaagcgcctacccttcggtcgctgcgctccctacgccccgccgcttcgcgtcggcctatcgcggccgctggccgctcaaaaatggctggcctacggccaggcaatctaccagggcgcggacaagccgcgccgtcgccactcgaccgccggcgcccacatcaaggcaccctgcctcgcgcgtttcggtgatgacggtgaaaacctctgacacatgcagctcccggagacggtcacagcttgtctgtaagcggatgccgggagcagacaagcccgtcagggcgcgtcagcgggtgttggcgggtgtcggggcgcagccatgacccagtcacgtagcgatagcggagtgtatactggcttaactatgcggcatcagagcagattgtactgagagtgcaccatatgcggtgtgaaataccgcacagatgcgtaaggagaaaataccgcatcaggcgctcttccgcttcctcgctcactgactcgctgcgctcggtcgttcggctgcggcgagcggtatcagctcactcaaaggcggtaatacggttatccacagaatcaggggataacgcaggaaagaacatgtgagcaaaaggccagcaaaaggccaggaaccgtaaaaaggccgcgttgctggcgtttttccataggctccgcccccctgacgagcatcacaaaaatcgacgctcaagtcagaggtggcgaaacccgacaggactataaagataccaggcgtttccccctggaagctccctcgtgcgctctcctgttccgaccctgccgcttaccggatacctgtccgcctttctcccttcgggaagcgtggcgctttctcatagctcacgctgtaggtatctcagttcggtgtaggtcgttcgctccaagctgggctgtgtgcacgaaccccccgttcagcccgaccgctgcgccttatccggtaactatcgtcttgagtccaacccggtaagacacgacttatcgccactggcagcagccactggtaacaggattagcagagcgaggtatgtaggcggtgctacagagttcttgaagtggtggcctaactacggctacactagaaggacagtatttggtatctgcgctctgctgaagccagttaccttcggaaaaagagttggtagctcttgatccggcaaacaaaccaccgctggtagcggtggtttttttgtttgcaagcagcagattacgcgcagaaaaaaaggatctcaagaagatcctttgatcttttctacggggtctgacgctcagtggaacgaaaactcacgttaagggattttggtcatgcatgatatatctcccaatttgtgtagggcttattatgcacgcttaaaaataataaaagcagacttgacctgatagtttggctgtgagcaattatgtgcttagtgcatctaatcgcttgagttaacgccggcgaagcggcgtcggcttgaacgaatttctagctagacattatttgccgactaccttggtgatctcgcctttcacgtagtggacaaattcttccaactgatctgcgcgcgaggccaagcgatcttcttcttgtccaagataagcctgtctagcttcaagtatgacgggctgatactgggccggcaggcgctccattgcccagtcggcagcgacatccttcggcgcgattttgccggttactgcgctgtaccaaatgcgggacaacgtaagcactacatttcgctcatcgccagcccagtcgggcggcgagttccatagcgttaaggtttcatttagcgcctcaaatagatcctgttcaggaaccggatcaaagagttcctccgccgctggacctaccaaggcaacgctatgttctcttgcttttgtcagcaagatagccagatcaatgtcgatcgtggctggctcgaagatacctgcaagaatgtcattgcgctgccattctccaaattgcagttcgcgcttagctggataacgccacggaatgatgtcgtcgtgcacaacaatggtgacttctacagcgcggagaatctcgctctctccaggggaagccgaagtttccaaaaggtcgttgatcaaagctcgccgcgttgtttcatcaagccttacggtcaccgtaaccagcaaatcaatatcactgtgtggcttcaggccgccatccactgcggagccgtacaaatgtacggccagcaacgtcggttcgagatggcgctcgatgacgccaactacctctgatagttgagtcgatacttcggcgatcaccgcttcccccatgatgtttaactttgttttagggcgactgccctgctgcgtaacatcgttgctgctccataacatcaaacatcgacccacggcgtaacgcgcttgctgcttggatgcccgaggcatagactgtaccccaaaaaaacatgtcataacaagaagccatgaaaaccgccactgcgccgttaccaccgctgcgttcggtcaaggttctggaccagttgcgtgacggcagttacgctacttgcattacagcttacgaaccgaacgaggcttatgtccactgggttcgtgcccgaattgatcacaggcagcaacgctctgtcatcgttacaatcaacatgctaccctccgcgagatcatccgtgtttcaaacccggcagcttagttgccgttcttccgaatagcatcggtaacatgagcaaagtctgccgccttacaacggctctcccgctgacgccgtcccggactgatgggctgcctgtatcgagtggtgattttgtgccgagctgccggtcggggagctgttggctggctggtggcaggatatattgtggtgtaaacaaattgacgcttagacaacttaataacacattgcggacgtttttaatgtactgaattaacgccgaattaattcgggggatctatagggactttaggtgatctggattttagtactggattttggttttaggaattagaaattttattgatagaagtattttacaaatacaaatacatactaagggtttcttatatgctcaacacgtgagcgaaaccctataagaaccctaattcccttatctgggaactactcacacattattatggagaaactcgatgtcgatcgactctagctagaggatcgatccgaaccccagagtcccgctcagaagaactcgtcaagaaggcgatagaaggcgatgcgctgcgaatcgggagcggcgataccgtaaagcacgaggaagcggtcagcccattcgccgccaagctcttcagcaatatcacgggtagccaacgctatgtcctgatagcggtccgccacacccagccggccacagtcgatgaatccagaaaagcggccattttccaccatgatattcggcaagcaggcatcgccatgtgtcacgacgagatcctcgccgtcgggcatgcgcgccttgagcctggcgaacagttcggctggcgcgagcccctgatgctcttcgtccagatcatcctgatcgacaagaccggcttccatccgagtacgtgctcgctcgatgcgatgtttcgcttggtggtcgaatgggcaggtagccggatcaagcgtatgcagccgccgcattgcatcagccatgatggatactttctcggcaggagcaaggtgagatgacaggagatcctgccccggcacttcgcccaatagcagccagtcccttcccgcttcagtgacaacgtcgagcacagctgcgcaaggaacgcccgtcgtggccagccacgatagccgcgctgcctcgtcctggagttcattcagggcaccggacaggtcggtcttgacaaaaagaaccgggcgcccctgcgctgacagccggaacacggcggcatcagagcagccgattgtctgttgtgcccagtcatagccgaatagcctctccacccaagcggccggagaacctgcgtgcaatccatcttgttcaatccccatggtcgatcgacagatctgcgaatcgagagagatagatttgtagagagagactggtgatttcagcgtgtcctctccaaatgaaatgaacttccttatatagaggaagggtcttgcgaaggatagtgggattgtgcgtcatcccttacgtcagtggagatatcacatcaatccacttgctttgaagacgtggttggaacgtcttctttttccacgatgctcctcgtgggtgggggtccatctttgggaccactgtcggcagaggcatcttgaacgatagcctttcctttatcgcaatgatggcatttgtaggtgccaccttccttttctactgtccttttgatgaagtgacagatagctgggcaatggaatccgaggaggtttcccgatattaccctttgttgaaaagtctcaatagccctttggtcttctgagactgtatctttgatattcttggagtagacgagagtgtcgtgctccaccatgttatcacatcaatccacttgctttgaagacgtggttggaacgtcttctttttccacgatgctcctcgtgggtgggggtccatctttgggaccactgtcggcagaggcatcttgaacgatagcctttcctttatcgcaatgatggcatttgtaggtgccaccttccttttctactgtccttttgatgaagtgacagatagctgggcaatggaatccgaggaggtttcccgatattaccctttgttgaaaagtctcaatagccctttggtcttctgagactgtatctttgatattcttggagtagacgagagtgtcgtgctccaccatgttggcaagctgctctagcattcgccattcaggctgcgcaactgttgggaagggcgatcggtgcgggcctcttcgctattacgccagctggcgaaagggggatgtgctgcaaggcgattaagttgggtaacgccagggttttcccagtcacgacgttgtaaaacgacggccagtgccaagcttgcatgcctgcaggtcaacatggtggagcacgacactctcgtctactccaagaatatcaaagatacagtctcagaagaccagagggctattgagacttttcaacaaagggtaatatcgggaaacctcctcggattccattgcccagctatctgtcacttcatcgaaaggacagtagaaaaggaagatggcttctacaaatgccatcattgcgataaaggaaaggctatcgttcaagatgcctctaccgacagtggtcccaaagatggacccccacccacgaggaacatcgtggaaaaagaagacgttccaaccacgtcttcaaagcaagtggattgatgtgatggtcaacatggtggagcacgacacacttgtctactccaaaaatatcaaagatacagtctcagaagaccaaagggcaattgagacttttcaacaaagggtaatatccggaaacctcctcggattccattgcccagctatctgtcactttattgtgaagatagtggaaaaggaaggtggctcctacaaatgccatcattgcgataaaggaaaggccatcgttgaagatgcctctgccgacagtggtcccaaagatggacccccacccacgaggagcatcgtggaaaaagaagacgttccaaccacgtcttcaaagcaagtggattgatgtgatatctccactgacgtaagggatgacgcacaatcccactatccttcgcaagacccttcctctatataaggaagttcatttcatttggagaggacctcgagaattctcaacacaacatatacaaaacaaacgaatctcaagcaatcaagcattctacttctattgcagcaatttaaatcatttcttttaaagcaaaagcaattttctgaaaattttcaccatttacgaacgatagccatggcaagggtgagcaagggcgaggagctgttcaccggggtggtgcccatcctggtcgagctggacggcgacgtaaacggccacaagttcagcgtgtccggcgagggcgagggcgatgccacctacggcaagctgaccctgaagttcatctgcaccaccggcaagctgcccgtgccctggcccaccctcgtgaccaccttcacctacggcgtgcagtgcttcagccgctaccccgaccacatgaagcagcacgacttcttcaagtccgccatgcccgaaggctacgtccaggagcgcaccatcttcttcaaggacgacggcaactacaagacccgcgccgaggtgaagttcgagggcgacaccctggtgaaccgcatcgagctgaagggcatcgacttcaaggaggacggcaacatcctggggcacaagctggagtacaactacaacagccacaacgtctatatcatggccgacaagcagaagaacggcatcaaggtgaacttcaagatccgccacaacatcgaggacggcagcgtgcagctcgccgaccactaccagcagaacacccccatcggcgacggccccgtgctgctgcccgacaaccactacctgagcacccagtccgccctgagcaaagaccccaacgagaagcgcgatcacatggtcctgctggagttcgtgaccgccgccgggatcactcacggcatggacgagctgtacaaggggatcctctagactagtcatcatcatcatcatcatgacaagcagaagaacggcatcaaggtgaacttcaagatccgccacaacatcgaggacggcagcgtgcagctcgccgaccactaccagcagaacacccccatcggcgacggccccgtgctgctgcccgacaaccactacctgagctaccagtccgccctgagcaaagaccccaacgagaagcgcgatcacatggtcctgctggagttcgtgaccgccgccgggatcactctcggcatggacgaactgtacaagtaacgcgttaatctagagtccgcaaaaatcaccagtctctctctacaaatctatctctctctatttttctccagaataatgtgtgagtagttcccagataagggaattagggttcttatagggtttcgctcatgtgttgagcatataagaaacccttagtatgtatttgtatttgtaaaatacttctatcaataaaatttctaattcctaaaaccaaaatccagtgacctgcaggcatgcaagcttgcatgcctgcaggtcgactctagaggatccccgggtaccgagctcgaattcgtaatcatggtcatagctgtttcctgtgtgaaattgttatccgctcacaattccacacaacatacgagccggaagcataaagtgtaaagcctggggtgcctaatgagtgagctaactcacattaattgcgttgcgctcactgcccgctttccagtcgggaaacctgtcgtgccagctgcattaatgaatcggccaacgcgcggggagaggcggtttgcgtattggctagagcagcttgagcttggatcagattgtcgtttcccgccttcagtttaaactatcagtgtttgacaggatatattggcgggtaaacctaagagaaaagagcgtttattagaataacggatatttaaaagggcgtgaaaaggtttatccgttcgtccatttgtatgtgcatgccaaccacagggttcccctcgggatcaa